European Patent Application EP 4 477 669 A1, published December 18, 2024. Title: ANTIGEN-BINDING MOLECULE SPECIFICALLY BINDING TO PSMA AND CD3, AND PHARMACEUTICAL USE THEREOF. Applicant: JIANGSU HENGRUI PHARMACEUTICALS CO., LTD. Application CN. The sequence listing filed with the application follows.

SEQUENCE LISTING (286 sequences)

SEQ ID NO: 1 - protein, 5 aa, Mus musculus
  REGION 1..5: note = 2-HCDR1
DYYMA

SEQ ID NO: 2 - protein, 17 aa, Mus musculus
  REGION 1..17: note = 2-HCDR2
NINFDGSSTYYLDSLKS

SEQ ID NO: 3 - protein, 11 aa, Mus musculus
  REGION 1..11: note = 2-HCDR3
DLDGYYGYFDV

SEQ ID NO: 4 - protein, 10 aa, Mus musculus
  REGION 1..10: note = 2-LCDR1
SASSSVSHMY

SEQ ID NO: 5 - protein, 7 aa, Mus musculus
  REGION 1..7: note = 2-LCDR2
RTSNLAS

SEQ ID NO: 6 - protein, 9 aa, Mus musculus
  REGION 1..9: note = 2-LCDR3
QQYHSYPLM

SEQ ID NO: 7 - protein, 5 aa, Mus musculus
  REGION 1..5: note = 13-HCDR1
NYAIS

SEQ ID NO: 8 - protein, 16 aa, Mus musculus
  REGION 1..16: note = 13-HCDR2
VIWTGGGTHYNSALKS

SEQ ID NO: 9 - protein, 16 aa, Mus musculus
  REGION 1..16: note = 13-HCDR3
KGNYYGSSLYYYAMNY

SEQ ID NO: 10 - protein, 11 aa, Mus musculus
  REGION 1..11: note = 13-LCDR1
RASQDISNYLN

SEQ ID NO: 11 - protein, 7 aa, Mus musculus
  REGION 1..7: note = 13-LCDR2
YTSRLQS

SEQ ID NO: 12 - protein, 9 aa, Mus musculus
  REGION 1..9: note = 13-LCDR3
QQGDTLPYT

SEQ ID NO: 13 - protein, 5 aa, Mus musculus
  REGION 1..5: note = 15-HCDR1
DHNMN

SEQ ID NO: 14 - protein, 17 aa, Mus musculus
  REGION 1..17: note = 15-HCDR2
LINPNYGTADYNQKFKG

SEQ ID NO: 15 - protein, 7 aa, Mus musculus
  REGION 1..7: note = 15-HCDR3
GSSLFAY

SEQ ID NO: 16 - protein, 11 aa, Mus musculus
  REGION 1..11: note = 15-LCDR1
KASQGVDTAVA

SEQ ID NO: 17 - protein, 7 aa, Mus musculus
  REGION 1..7: note = 15-LCDR2
WASTRHT

SEQ ID NO: 18 - protein, 9 aa, Mus musculus
  REGION 1..9: note = 15-LCDR3
QQYSRYPLT

SEQ ID NO: 19 - protein, 5 aa, Mus musculus
  REGION 1..5: note = 19-HCDR1
DYYMA

SEQ ID NO: 20 - protein, 17 aa, Mus musculus
  REGION 1..17: note = 19-HCDR2
NINYDGSSTYYLDSLKS

SEQ ID NO: 21 - protein, 10 aa, Mus musculus
  REGION 1..10: note = 19-HCDR3
GGDYWDAMDY

SEQ ID NO: 22 - protein, 11 aa, Mus musculus
  REGION 1..11: note = 19-LCDR1
RASQDISKYLN

SEQ ID NO: 23 - protein, 7 aa, Mus musculus
  REGION 1..7: note = 19-LCDR2
YTSSLHS

SEQ ID NO: 24 - protein, 9 aa, Mus musculus
  REGION 1..9: note = 19-LCDR3
QQGNRLPRT

SEQ ID NO: 25 - protein, 5 aa, Mus musculus
  REGION 1..5: note = 27-HCDR1
DYYMA

SEQ ID NO: 26 - protein, 17 aa, Mus musculus
  REGION 1..17: note = 27-HCDR2
NINYDGSSTYYLDSLKS

SEQ ID NO: 27 - protein, 11 aa, Mus musculus
  REGION 1..11: note = 27-HCDR3
DLDGYYGYFDV

SEQ ID NO: 28 - protein, 10 aa, Mus musculus
  REGION 1..10: note = 27-LCDR1
SASSSVSYMY

SEQ ID NO: 29 - protein, 7 aa, Mus musculus
  REGION 1..7: note = 27-LCDR2
RTSNLAS

SEQ ID NO: 30 - protein, 9 aa, Mus musculus
  REGION 1..9: note = 27-LCDR3
QQYHSYPLT

SEQ ID NO: 31 - protein, 5 aa, Mus musculus
  REGION 1..5: note = 31-HCDR1
DYYMA

SEQ ID NO: 32 - protein, 17 aa, Mus musculus
  REGION 1..17: note = 31-HCDR2
SINYDGSSTYYLDSLKS

SEQ ID NO: 33 - protein, 10 aa, Mus musculus
  REGION 1..10: note = 31-HCDR3
SDGYWAWFAY

SEQ ID NO: 34 - protein, 11 aa, Mus musculus
  REGION 1..11: note = 31-LCDR1
RASGNIHNYLA

SEQ ID NO: 35 - protein, 7 aa, Mus musculus
  REGION 1..7: note = 31-LCDR2
NAETLAD

SEQ ID NO: 36 - protein, 9 aa, Mus musculus
  REGION 1..9: note = 31-LCDR3
QHFWSTPPT

SEQ ID NO: 37 - protein, 5 aa, Mus musculus
  REGION 1..5: note = 41-HCDR1
SYGIS

SEQ ID NO: 38 - protein, 17 aa, Mus musculus
  REGION 1..17: note = 41-HCDR2
EIFPRRGNTYYNEKFRG

SEQ ID NO: 39 - protein, 12 aa, Mus musculus
  REGION 1..12: note = 41-HCDR3
VFDGYYNYAMDY

SEQ ID NO: 40 - protein, 11 aa, Mus musculus
  REGION 1..11: note = 41-LCDR1
RASQDIGSSLN

SEQ ID NO: 41 - protein, 7 aa, Mus musculus
  REGION 1..7: note = 41-LCDR2
ATSSLDS

SEQ ID NO: 42 - protein, 9 aa, Mus musculus
  REGION 1..9: note = 41-LCDR3
LQYASSPYT

SEQ ID NO: 43 - protein, 5 aa, Mus musculus
  REGION 1..5: note = 43-HCDR1
NYWMN

SEQ ID NO: 44 - protein, 19 aa, Mus musculus
  REGION 1..19: note = 43-HCDR2
QVRLKSDNYATHYAESVKG

SEQ ID NO: 45 - protein, 11 aa, Mus musculus
  REGION 1..11: note = 43-HCDR3
NYYGPAGPFDF

SEQ ID NO: 46 - protein, 11 aa, Mus musculus
  REGION 1..11: note = 43-LCDR1
KASQNVHTSVA

SEQ ID NO: 47 - protein, 7 aa, Mus musculus
  REGION 1..7: note = 43-LCDR2
SASNRYS

SEQ ID NO: 48 - protein, 9 aa, Mus musculus
  REGION 1..9: note = 43-LCDR3
QQYSSYPLT

SEQ ID NO: 49 - protein, 5 aa, Mus musculus
  REGION 1..5: note = 46-HCDR1
NYGMS

SEQ ID NO: 50 - protein, 17 aa, Mus musculus
  REGION 1..17: note = 46-HCDR2
TIGSGGGYTYYSDSVKG

SEQ ID NO: 51 - protein, 6 aa, Mus musculus
  REGION 1..6: note = 46-HCDR3
HPQIGY

SEQ ID NO: 52 - protein, 11 aa, Mus musculus
  REGION 1..11: note = 46-LCDR1
KASQSVGTAVA

SEQ ID NO: 53 - protein, 7 aa, Mus musculus
  REGION 1..7: note = 46-LCDR2
SASSRYT

SEQ ID NO: 54 - protein, 9 aa, Mus musculus
  REGION 1..9: note = 46-LCDR3
HQYSSYPLT

SEQ ID NO: 55 - protein, 5 aa, Mus musculus
  REGION 1..5: note = 50-HCDR1
NYGIS

SEQ ID NO: 56 - protein, 17 aa, Mus musculus
  REGION 1..17: note = 50-HCDR2
EIYPRSGNTYYNTNFKG

SEQ ID NO: 57 - protein, 12 aa, Mus musculus
  REGION 1..12: note = 50-HCDR3
NPFTTVVEGFAF

SEQ ID NO: 58 - protein, 16 aa, Mus musculus
  REGION 1..16: note = 50-LCDR1
RSSQSILHSNGNTYLE

SEQ ID NO: 59 - protein, 7 aa, Mus musculus
  REGION 1..7: note = 50-LCDR2
RVSNRFS

SEQ ID NO: 60 - protein, 9 aa, Mus musculus
  REGION 1..9: note = 50-LCDR3
FQGLHVPPT

SEQ ID NO: 61 - protein, 5 aa, Mus musculus
  REGION 1..5: note = 71-HCDR1
NYRMH

SEQ ID NO: 62 - protein, 19 aa, Mus musculus
  REGION 1..19: note = 71-HCDR2
VITVKSDNYGSSYAESVKG

SEQ ID NO: 63 - protein, 8 aa, Mus musculus
  REGION 1..8: note = 71-HCDR3
ELGQVLVF

SEQ ID NO: 64 - protein, 16 aa, Mus musculus
  REGION 1..16: note = 71-LCDR1
RSSQSLVHSYGNTYLH

SEQ ID NO: 65 - protein, 7 aa, Mus musculus
  REGION 1..7: note = 71-LCDR2
KVSNRFS

SEQ ID NO: 66 - protein, 9 aa, Mus musculus
  REGION 1..9: note = 71-LCDR3
SQTTHVPWT

SEQ ID NO: 67 - protein, 5 aa, Mus musculus
  REGION 1..5: note = 73-HCDR1
TSWMN

SEQ ID NO: 68 - protein, 17 aa, Mus musculus
  REGION 1..17: note = 73-HCDR2
RIYPGDGDTKYNGKFQG

SEQ ID NO: 69 - protein, 10 aa, Mus musculus
  REGION 1..10: note = 73-HCDR3
SIYYLYYFDY

SEQ ID NO: 70 - protein, 11 aa, Mus musculus
  REGION 1..11: note = 73-LCDR1
STSQDIYNNLS

SEQ ID NO: 71 - protein, 7 aa, Mus musculus
  REGION 1..7: note = 73-LCDR2
YTSSLHS

SEQ ID NO: 72 - protein, 9 aa, Mus musculus
  REGION 1..9: note = 73-LCDR3
QQYNNLPFT

SEQ ID NO: 73 - protein, 120 aa, Mus musculus
  REGION 1..120: note = 2
EVKLVESEGGLVQPGSSMKLSCTASGFTFSDYYMAWVRQVPEKGLEWVANINFDGSSTYYLDSLKSRFIISRDNAKNILYLQMSSLKSEDTATYYCARDLDGYYGYFDVWGTGTTVTVSS

SEQ ID NO: 74 - protein, 106 aa, Mus musculus
  REGION 1..106: note = 2
QIVLTQSPAIMSASPGEKVTISCSASSSVSHMYWYQQKPGSSPKPWIYRTSNLASGVPARFSGSGSGTSYSLTISSMEAEDAATYYCQQYHSYPLMFGAGTKLELK

SEQ ID NO: 75 - protein, 128 aa, Mus musculus
  REGION 1..128: note = 13
QVQLKESGPGLVAPSQSLSITCTVSGFSLTNYAISWVRQPPGKGLEWLGVIWTGGGTHYNSALKSRLSISKDNSKSQVFLKMNSLQTDDTARYYCARKGNYYGSSLYYYAMNYWGQGTSVTVSSTVSS

SEQ ID NO: 76 - protein, 106 aa, Mus musculus
  REGION 1..106: note = 13
DIQMTQTTSSLSASLGDRVTISCRASQDISNYLNWYQQKPDGTVKLLIYYTSRLQSGVPSRFSGSGSGTDYSLSISNLEQEDIATYFCQQGDTLPYTFGGGTKLEI

SEQ ID NO: 77 - protein, 116 aa, Mus musculus
  REGION 1..116: note = 15
EFQLQQSGPELVKPGASVKISCKASGYSFTDHNMNWVKQSNGKSLEWIGLINPNYGTADYNQKFKGKATLTVDQSSTTAFMQFTSLTSEDSAVYYCARGSSLFAYWGQGTLVTVSA

SEQ ID NO: 78 - protein, 107 aa, Mus musculus
  REGION 1..107: note = 15
DIVMTQSHKFMSTSVGDRVNITCKASQGVDTAVAWYQQKPGQSPKLLIYWASTRHTGVPDRFTGSGSGTDFTLTISNVQSEDLADYFCQQYSRYPLTFGAGTKLELK

SEQ ID NO: 79 - protein, 119 aa, Mus musculus
  REGION 1..119: note = 19
EVKLVESEGGLVQPGSSMKLSCTASGFTFSDYYMAWVRQVPERGLEWVANINYDGSSTYYLDSLKSRFIISRDNAKNILYLQMSSLKSEDTATYYCARGGDYWDAMDYWGQGTSVTVSS

SEQ ID NO: 80 - protein, 107 aa, Mus musculus
  REGION 1..107: note = 19
DIQMTQTTSSLSASLGDRVTISCRASQDISKYLNWYQQKPDGTVKLLIYYTSSLHSGVPSRFSGSGSGTDYSLTISNLEQEDIATYFCQQGNRLPRTFGGGTKLEIK

SEQ ID NO: 81 - protein, 120 aa, Mus musculus
  REGION 1..120: note = 27
EVKLVESEGGLVQPGSSMKLSCTASGFTFSDYYMAWVRQVPEKGLEWVANINYDGSSTYYLDSLKSRFIISRDNAKNILYLQMSSLKSEDTATYYCARDLDGYYGYFDVWGTGTTVTVSS

SEQ ID NO: 82 - protein, 106 aa, Mus musculus
  REGION 1..106: note = 27
QIVLTQSPAIMSASPGEKVTISCSASSSVSYMYWYQQKPGSSPKPWIYRTSNLASGVPARFSGSGSGTSYSLTISSMEAEDAATYYCQQYHSYPLTFGAGTKLELK

SEQ ID NO: 83 - protein, 119 aa, Mus musculus
  REGION 1..119: note = 31
EVKLVESEGGLVQPGSSKKLSCTASGFTFSDYYMAWVRQVPEKGLEWVASINYDGSSTYYLDSLKSRFIISRDNAKNNLYLQMNSLKSEDTATYYCAGSDGYWAWFAYWGQGTLVTVSA

SEQ ID NO: 84 - protein, 107 aa, Mus musculus
  REGION 1..107: note = 31
DIQMTQSPASLSASVGEAVTITCRASGNIHNYLAWYQQKQGKSPQLLVYNAETLADGVPSRFSGSGSGTQFSLKINSLRPEDFGSYYCQHFWSTPPTFGGGTKLEIK

SEQ ID NO: 85 - protein, 121 aa, Mus musculus
  REGION 1..121: note = 41
QVQLQQSGAELARPGASVKLSCKASGYTFTSYGISWVKQRTGQGLEWIGEIFPRRGNTYYNEKFRGKATLTADKSSSAAYMELRSLTSEDSAVYFCARVFDGYYNYAMDYWGQGTSVTVSS

SEQ ID NO: 86 - protein, 107 aa, Mus musculus
  REGION 1..107: note = 41
DIQMTQSPSSLSASLGERVSLTCRASQDIGSSLNWLQQQPDGTIKRLIYATSSLDSGVPTRFSGSRSGSDYSLTISSLESEDFVDYYCLQYASSPYTFGGGTKLEIK

SEQ ID NO: 87 - protein, 122 aa, Mus musculus
  REGION 1..122: note = 43
EVKFEESGGGLVQPGGSMKLSCVASGFTFSNYWMNWLRQSPEKGLEWVAQVRLKSDNYATHYAESVKGRFTISRDDSKSSAYLQMNNLRAEDTGIYYCSENYYGPAGPFDFWGQGTTLTVSS

SEQ ID NO: 88 - protein, 107 aa, Mus musculus
  REGION 1..107: note = 43
DIVMTQSQKFMSTTVGDRVSITCKASQNVHTSVAWYQQKPGQSPKLLIYSASNRYSGVPDRFTGSGSGTDFTLTINNMQSEDLADYFCQQYSSYPLTFGVGTKLELK

SEQ ID NO: 89 - protein, 115 aa, Mus musculus
  REGION 1..115: note = 46
EVQLVESGGDLVKPGGSLKLSCAASGFTFSNYGMSWVRQTPDKRIKWVATIGSGGGYTYYSDSVKGRFTISRDNAKNTLYLQMSSLKSEDTAIYYCVRHPQIGYWGQGTLVTVSA

SEQ ID NO: 90 - protein, 107 aa, Mus musculus
  REGION 1..107: note = 46
DIVMTQSQKFMSTTVGDRVTITCKASQSVGTAVAWYQQKPGQSPKLLIYSASSRYTGVPDRFTGSGSGTDFTLTITNMQSEDLADYFCHQYSSYPLTFGGGTKLEIK

SEQ ID NO: 91 - protein, 121 aa, Mus musculus
  REGION 1..121: note = 50
QVQLQQSGAELARPGASVKLSCKASGFTFTNYGISWVKQRTGQGLEWIGEIYPRSGNTYYNTNFKGEATLTADKSSSTAFMELRSLTSEDSAVYFCARNPFTTVVEGFAFWGQGTLVTVSA

SEQ ID NO: 92 - protein, 112 aa, Mus musculus
  REGION 1..112: note = 50
DVFMTQSPLSLPVSLGDQASISCRSSQSILHSNGNTYLEWYLQKPGQSPKLLIYRVSNRFSGVPDRFSGSGSGTDFTLKISRVEAEDLGVYYCFQGLHVPPTFGAGTKLELK

SEQ ID NO: 93 - protein, 119 aa, Mus musculus
  REGION 1..119: note = 71
QVQLVETGGGLVRPGNSLKLSCVTSGFTFSNYRMHWLRQPPGKRLEWIAVITVKSDNYGSSYAESVKGRFAISRDDSKSSVYLEMNRLREEDTATYFCSRELGQVLVFWGQGTLVTVSA

SEQ ID NO: 94 - protein, 112 aa, Mus musculus
  REGION 1..112: note = 71
DVVVTQTPLSLPVSLGDQASISCRSSQSLVHSYGNTYLHWYLQKPGQSPKLLIYKVSNRFSGVPDRFSGSGSGTDFTLKISRVEAEDLGVYFCSQTTHVPWTFGGGTKLEIK

SEQ ID NO: 95 - protein, 119 aa, Mus musculus
  REGION 1..119: note = 73
QVQLQQSGPELVKPGASVKISCKASGYAFSTSWMNWVKERPGKGLEWIGRIYPGDGDTKYNGKFQGKATLTADKSSSTAYMKLSSLTSEDSAVYFCVRSIYYLYYFDYWGQGTTLTVSS

SEQ ID NO: 96 - protein, 107 aa, Mus musculus
  REGION 1..107: note = 73
DIQMTQPTSSLSASLGDRVTISCSTSQDIYNNLSWFQQKPDGTVRLLIYYTSSLHSGVPSRFSGSGSGTDYSLTISNLEPEDIATYYCQQYNNLPFTFGGGTNLEIR

SEQ ID NO: 97 - protein, 330 aa, synthetic construct [sequence omitted]

SEQ ID NO: 98 - protein, 107 aa, synthetic construct [sequence omitted]

SEQ ID NO: 99 - protein, 120 aa, synthetic construct
  REGION 1..120: note = hu2H1
EVQLVESGGGLVQPGGSLRLSCAASGFTFSDYYMAWVRQAPGKGLEWVANINFDGSSTYYLDSLKSRFTISRDNAKNSLYLQMNSLRAEDTAVYYCARDLDGYYGYFDVWGQGTTVTVSS

SEQ ID NO: 100 - protein, 106 aa, synthetic construct
  REGION 1..106: note = hu2L1
EIVLTQSPDFQSVTPKEKVTITCSASSSVSHMYWYQQKPDQSPKLLIYRTSNLASGVPSRFSGSGSGTDFTLTINSLEAEDAATYYCQQYHSYPLMFGQGTKLEIK

SEQ ID NO: 101 - protein, 124 aa, synthetic construct
  REGION 1..124: note = hu13H1
EVTLKESGPVLVKPTETLTLTCTVSGFSLSNYAISWIRQPPGKALEWLAVIWTGGGTHYNSALKSRLTISKDTSKSQVVLTMTNMDPVDTATYYCARKGNYYGSSLYYYAMNYWGQGTTVTVSS

SEQ ID NO: 102 - protein, 124 aa, synthetic construct
  REGION 1..124: note = hu13H2
EVTLKESGPVLVKPTETLTLTCTVSGFSLSNYAISWIRQPPGKALEWLGVIWTGGGTHYNSALKSRLTISKDTSKSQVVLTMTNMDPVDTARYYCARKGNYYGSSLYYYAMNYWGQGTTVTVSS

SEQ ID NO: 103 - protein, 124 aa, synthetic construct
  REGION 1..124: note = hu13H3
EVTLKESGPVLVKPTETLTLTCTVSGFSLTNYAISWIRQPPGKGLEWLGVIWTGGGTHYNSALKSRLTISKDNSKSQVVLTMTNMDPVDTARYYCARKGNYYGSSLYYYAMNYWGQGTTVTVSS

SEQ ID NO: 104 - protein, 107 aa, synthetic construct
  REGION 1..107: note = hu13L1
DIQMTQSPSSLSASVGDRVTITCRASQDISNYLNWYQQKPGKAPKLLIYYTSRLQSGVPSRFSGSGSGTDFTLTISSLQPEDFATYYCQQGDTLPYTFGGGTKVEIK

SEQ ID NO: 105 - protein, 107 aa, synthetic construct
  REGION 1..107: note = hu13L2
DIQMTQSPSSLSASVGDRVTITCRASQDISNYLNWYQQKPDGAPKLLIYYTSRLQSGVPSRFSGSGSGTDYTLTISSLQPEDFATYYCQQGDTLPYTFGGGTKVEIK

SEQ ID NO: 106 - protein, 107 aa, synthetic construct
  REGION 1..107: note = hu13L3
DIQMTQSPSSLSASVGDRVTITCRASQDISNYLNWYQQKPDGTVKLLIYYTSRLQSGVPSRFSGSGSGTDYTLTISSLQPEDFATYYCQQGDTLPYTFGGGTKVEIK

SEQ ID NO: 107 - protein, 116 aa, synthetic construct
  REGION 1..116: note = hu15H1
EFQLVQSGAEVKKPGASVKVSCKASGYTFTDHNMNWVRQAPGQRLEWMGLINPNYGTADYNQKFKGRVTITRDTSASTAYMELSSLRSEDTAVYYCARGSSLFAYWGQGTLVTVSS

SEQ ID NO: 108 - protein, 116 aa, synthetic construct
  REGION 1..116: note = hu15H2
EFQLVQSGAEVKKPGASVKVSCKASGYSFTDHNMNWVRQAPGQRLEWMGLINPNYGTADYNQKFKGRVTITRDTSASTAYMELSSLRSEDTAVYYCARGSSLFAYWGQGTLVTVSS

SEQ ID NO: 109 - protein, 116 aa, synthetic construct
  REGION 1..116: note = hu15H3
EFQLVQSGAEVKKPGASVKVSCKASGYSFTDHNMNWVRQAPGQRLEWMGLINPNYGTADYNQKFKGRVTITVDQSASTAYMELSSLRSEDTAVYYCARGSSLFAYWGQGTLVTVSS

SEQ ID NO: 110 - protein, 116 aa, synthetic construct
  REGION 1..116: note = hu15H4
EFQLVQSGAEVKKPGASVKVSCKASGYSFTDHNMNWVRQAPGQRLEWMGLINPNYGTADYNQKFKGRVTLTVDQSATTAYMELSSLRSEDTAVYYCARGSSLFAYWGQGTLVTVSS

SEQ ID NO: 111 - protein, 116 aa, synthetic construct
  REGION 1..116: note = hu15H5
EFQLVQSGAEVKKPGASVKVSCKASGYSFTDHNMNWVRQAPGQRLEWIGLINPNYGTADYNQKFKGRATLTVDQSATTAYMELSSLRSEDTAVYYCARGSSLFAYWGQGTLVTVSS

SEQ ID NO: 112 - protein, 116 aa, synthetic construct
  REGION 1..116: note = hu15H6
EFQLVQSGAEVKKPGASVKVSCKASGYSFTDHNMNWVRQAPGQCLEWMGLINPNYGTADYNQKFKGRVTLTVDQSATTAYMELSSLRSEDTAVYYCARGSSLFAYWGQGTLVTVSS

SEQ ID NO: 113 - protein, 107 aa, synthetic construct
  REGION 1..107: note = hu15L1
DIQMTQSPSSLSASVGDRVTITCKASQGVDTAVAWYQQKPGKVPKLLIYWASTRHTGVPSRFSGSGSGTDFTLTISSLQPEDVATYYCQQYSRYPLTFGQGTKLEIK

SEQ ID NO: 114 - protein, 107 aa, synthetic construct
  REGION 1..107: note = hu15L2
DIQMTQSPSSLSASVGDRVTITCKASQGVDTAVAWYQQKPGKSPKLLIYWASTRHTGVPDRFSGSGSGTDFTLTISSLQPEDVATYYCQQYSRYPLTFGQGTKLEIK

SEQ ID NO: 115 - protein, 107 aa, synthetic construct
  REGION 1..107: note = hu15L3
DIQMTQSPSSLSASVGDRVTITCKASQGVDTAVAWYQQKPGKSPKLLIYWASTRHTGVPDRFSGSGSGTDFTLTISSLQPEDVATYYCQQYSRYPLTFGCGTKLEIK

SEQ ID NO: 116 - protein, 119 aa, synthetic construct
  REGION 1..119: note = hu19H1
EVQLVESGGGLVQPGGSLRLSCAASGFTFSDYYMAWVRQAPGKGLEWVANINYDGSSTYYLDSLKSRFTISRDNAKNSLYLQMNSLRAEDTAVYYCARGGDYWDAMDYWGQGTTVTVSS

SEQ ID NO: 117 - protein, 119 aa, synthetic construct
  REGION 1..119: note = hu19H2
EVKLVESGGGLVQPGGSLRLSCAASGFTFSDYYMAWVRQAPGKGLEWVANINYDGSSTYYLDSLKSRFTISRDNAKNSLYLQMNSLRAEDTAVYYCARGGDYWDAMDYWGQGTTVTVSS

SEQ ID NO: 118 - protein, 107 aa, synthetic construct
  REGION 1..107: note = hu19L1
DIQMTQSPSSLSASVGDRVTITCRASQDISKYLNWYQQKPGKAPKLLIYYTSSLHSGVPSRFSGSGSGTDFTLTISSLQPEDFATYYCQQGNRLPRTFGGGTKVEIK

SEQ ID NO: 119 - protein, 107 aa, synthetic construct
  REGION 1..107: note = hu19L2
DIQMTQSPSSLSASVGDRVTITCRASQDISKYLNWYQQKPGKAPKLLIYYTSSLHSGVPSRFSGSGSGTDYTLTISSLQPEDFATYYCQQGNRLPRTFGGGTKVEIK

SEQ ID NO: 120 - protein, 120 aa, synthetic construct
  REGION 1..120: note = hu27H1
EVQLVESGGGLVQPGGSLRLSCAASGFTFSDYYMAWVRQAPGKGLEWVANINYDGSSTYYLDSLKSRFTISRDNAKNSLYLQMNSLRAEDTAVYYCARDLDGYYGYFDVWGQGTTVTVSS

SEQ ID NO: 121 - protein, 106 aa, synthetic construct
  REGION 1..106: note = hu27L1
EIVLTQSPDFQSVTPKEKVTITCSASSSVSYMYWYQQKPDQSPKPWIYRTSNLASGVPSRFSGSGSGTDFTLTINSLEAEDAATYYCQQYHSYPLTFGQGTKLEIK

SEQ ID NO: 122 - protein, 106 aa, synthetic construct
  REGION 1..106: note = hu27L2
EIVLTQSPDFQSVTPKEKVTITCSASSSVSYMYWYQQKPDQSPKPWIYRTSNLASGVPSRFSGSGSGTDYTLTINSLEAEDAATYYCQQYHSYPLTFGQGTKLEIK

SEQ ID NO: 123 - protein, 106 aa, synthetic construct
  REGION 1..106: note = hu27L3
QIVLTQSPDFQSVTPKEKVTITCSASSSVSYMYWYQQKPDQSPKPWIYRTSNLASGVPSRFSGSGSGTDYTLTINSLEAEDAATYYCQQYHSYPLTFGQGTKLEIK

SEQ ID NO: 124 - protein, 106 aa, synthetic construct
  REGION 1..106: note = hu27L4
EIVLTQSPDFQSVTPKEKVTIQCSASSSVSYMYWYQQKPDQSPKPWIYRTSNLASGVPSRFSGSGSGTDFTLTINSLEAEDAATYYCQQYHSYPLTFGQGTKLEIK

SEQ ID NO: 125 - protein, 106 aa, synthetic construct
  REGION 1..106: note = hu27L5
EIVLTQSPDFQSVTPKEKVTIQCSASSSVSYMYWYQQKPDQSPKPWIYRTSNLASGVPSRFSGSGSGTDYTLTINSLEAEDAATYYCQQYHSYPLTFGQGTKLEIK

SEQ ID NO: 126 - protein, 106 aa, synthetic construct
  REGION 1..106: note = hu27L6
QIVLTQSPDFQSVTPKEKVTIQCSASSSVSYMYWYQQKPDQSPKPWIYRTSNLASGVPSRFSGSGSGTDYTLTINSLEAEDAATYYCQQYHSYPLTFGQGTKLEIK

SEQ ID NO: 127 - protein, 119 aa, synthetic construct
  REGION 1..119: note = hu31H1
EVQLVESGGGLVQPGGSLRLSCAASGFTFSDYYMAWVRQAPGKGLEWVASINYDGSSTYYLDSLKSRFTISRDNAKNSLYLQMNSLRAEDTAVYYCAGSDGYWAWFAYWGQGTLVTVSS

SEQ ID NO: 128 - protein, 107 aa, synthetic construct
  REGION 1..107: note = hu31L1
DIQMTQSPSSLSASVGDRVTITCRASGNIHNYLAWYQQKPGKAPKLLIYNAETLADGVPSRFSGSGSGTDFTLTISSLQPEDFATYYCQHFWSTPPTFGGGTKVEIK

SEQ ID NO: 129 - protein, 107 aa, synthetic construct
  REGION 1..107: note = hu31L2
DIQMTQSPSSLSASVGDRVTITCRASGNIHNYLAWYQQKPGKAPQLLVYNAETLADGVPSRFSGSGSGTDFTLTISSLQPEDFATYYCQHFWSTPPTFGGGTKVEIK

SEQ ID NO: 130 - protein, 107 aa, synthetic construct
  REGION 1..107: note = hu31L3
DIQMTQSPSSLSASVGDRVTITCRASGNIHNYLAWYQQKPGKSPQLLVYNAETLADGVPSRFSGSGSGTQFTLTISSLQPEDFATYYCQHFWSTPPTFGGGTKVEIK

SEQ ID NO: 131 - protein, 121 aa, synthetic construct
  REGION 1..121: note = hu41H1
EVQLVQSGAEVKKPGASVKVSCKASGYTFTSYGISWVRQAPGQGLEWMGEIFPRRGNTYYNEKFRGRVTMTTDKSTSTAYMELRSLRSDDTAVYYCARVFDGYYNYAMDYWGQGTTVTVSS

SEQ ID NO: 132 - protein, 121 aa, synthetic construct
  REGION 1..121: note = hu41H2
EVQLVQSGAEVKKPGASVKVSCKASGYTFTSYGISWVRQAPGQGLEWMGEIFPRRGNTYYNEKFRGRVTLTADKSTSTAYMELRSLRSDDTAVYYCARVFDGYYNYAMDYWGQGTTVTVSS

SEQ ID NO: 133 - protein, 107 aa, synthetic construct
  REGION 1..107: note = hu41L1
DIQMTQSPSSLSASVGDRVTITCRASQDIGSSLNWLQQKPGKAPKRLIYATSSLDSGVPSRFSGSRSGTDFTLTISSLQPEDFATYYCLQYASSPYTFGGGTKVEIK

SEQ ID NO: 134 - protein, 107 aa, synthetic construct
  REGION 1..107: note = hu41L2
DIQMTQSPSSLSASVGDRVTITCRASQDIGSSLNWLQQKPGKAIKRLIYATSSLDSGVPSRFSGSRSGTDYTLTISSLQPEDFATYYCLQYASSPYTFGGGTKVEIK

SEQ ID NO: 135 - protein, 107 aa, synthetic construct
  REGION 1..107: note = hu41L3
DIQMTQSPSSLSASVGDRVTITCRASQDIGSSLNWLQQKPGGAIKRLIYATSSLDSGVPSRFSGSRSGSDYTLTISSLQPEDFATYYCLQYASSPYTFGGGTKVEIK

SEQ ID NO: 136 - protein, 122 aa, synthetic construct
  REGION 1..122: note = hu43H1
EVQFVESGGGLVQPGGSLRLSCAASGFTFSNYWMNWVRQAPGKGLEWVAQVRLKSDNYATHYAESVKGRFTISRDNAKNSAYLQMNSLRAEDTAVYYCSENYYGPAGPFDFWGQGTTVTVSS

SEQ ID NO: 137 - protein, 122 aa, synthetic construct
  REGION 1..122: note = hu43H2
EVQFVESGGGLVQPGGSLRLSCAASGFTFSNYWMNWVRQAPGKGLEWVAQVRLKSDNYATHYAESVKGRFTISREDAKNSAYLQMNSLRAEDTAVYYCSENYYGPAGPFDFWGQGTTVTVSS

SEQ ID NO: 138 - protein, 122 aa, synthetic construct
  REGION 1..122: note = hu43H3
EVQFVESGGGLVQPGGSLRLSCAASGFTFSNYWMNWLRQAPGKGLEWVAQVRLKSDNYATHYAESVKGRFTISREDAKNSAYLQMNSLRAEDTAVYYCSENYYGPAGPFDFWGQGTTVTVSS

SEQ ID NO: 139 - protein, 107 aa, synthetic construct
  REGION 1..107: note = hu43L1
DIQMTQSPSSVSASVGDRVTITCKASQNVHTSVAWYQQKPGKSPKLLIYSASNRYSGVPSRFSGSGSGTDFTLTISSLQPEDFATYYCQQYSSYPLTFGQGTKLEIK

SEQ ID NO: 140 - protein, 107 aa, synthetic construct
  REGION 1..107: note = hu43L2
DIQMTQSPSSLSASVGDRVTITCKASQNVHTSVAWYQQKPGKSPKLLIYSASNRYSGVPSRFSGSGSGTDFTLTISSLQPEDVATYYCQQYSSYPLTFGQGTKLEIK

SEQ ID NO: 141 - protein, 115 aa, synthetic construct
  REGION 1..115: note = hu46H1
EVQLVESGGGLVKPGGSLRLSCAASGFTFSNYGMSWVRQAPGKGLEWVSTIGSGGGYTYYSDSVKGRFTISRDNAKNSLYLQMNSLRAEDTAVYYCARHPQIGYWGQGTLVTVSS

SEQ ID NO: 142 - protein, 115 aa, synthetic construct
  REGION 1..115: note = hu46H2
EVQLVESGGGLVKPGGSLRLSCAASGFTFSNYGMSWVRQAPGKGLEWVSTIGSGGGYTYYSDSVKGRFTISRDNAKNSLYLQMNSLRAEDTAVYYCVRHPQIGYWGQGTLVTVSS

SEQ ID NO: 143 - protein, 115 aa, synthetic construct
  REGION 1..115: note = hu46H3
EVQLVESGGGLVKPGGSLRLSCAASGFTFSNYGMSWVRQAPGKGIKWVSTIGSGGGYTYYSDSVKGRFTISRDNAKNSLYLQMNSLRAEDTAVYYCVRHPQIGYWGQGTLVTVSS

SEQ ID NO: 144 - protein, 115 aa, synthetic construct
  REGION 1..115: note = hu46H4
EVQLVESGGGLVKPGGSLRLSCAASGFTFSNYGMSWVRQAPGKGIKWVATIGSGGGYTYYSDSVKGRFTISRDNAKNSLYLQMNSLRAEDTAVYYCVRHPQIGYWGQGTLVTVSS

SEQ ID NO: 145 - protein, 107 aa, synthetic construct
  REGION 1..107: note = hu46L1
DIQMTQSPSSLSASVGDRVTITCKASQSVGTAVAWYQQKPGKAPKLLIYSASSRYTGVPSRFSGSGSGTDFTLTISSLQPEDFATYYCHQYSSYPLTFGGGTKVEIK

SEQ ID NO: 146 - protein, 107 aa, synthetic construct
  REGION 1..107: note = hu46L2
DIQMTQSPSSLSASVGDRVTITCKASQSVGTAVAWYQQKPGKAPKLLIYSASSRYTGVPSRFSGSGSGTDFTLTISSLQPEDFADYFCHQYSSYPLTFGGGTKVEIK

SEQ ID NO: 147 - protein, 107 aa, synthetic construct
  REGION 1..107: note = hu46L3
DIQMTQSPSSLSASVGDRVTITCKASQSVGTAVAWYQQKPGKAPKLLIYSASSRYTGVPDRFSGSGSGTDFTLTISSLQPEDFADYFCHQYSSYPLTFGGGTKVEIK

SEQ ID NO: 148 - protein, 121 aa, synthetic construct
  REGION 1..121: note = hu50H1
EVQLVQSGAEVKKPGASVKVSCKASGFTFTNYGISWVRQAPGQGLEWMGEIYPRSGNTYYNTNFKGRVTMTTDKSTSTAYMELRSLRSEDTAVYYCARNPFTTVVEGFAFWGQGTLVTVSS

SEQ ID NO: 149 - protein, 121 aa, synthetic construct
  REGION 1..121: note = hu50H2
EVQLVQSGAEVKKPGASVKVSCKASGFTFTNYGISWVRQAPGQGLEWMGEIYPRSGNTYYNTNFKGRVTLTADKSTSTAYMELRSLRSEDTAVYYCARNPFTTVVEGFAFWGQGTLVTVSS

SEQ ID NO: 150 - protein, 112 aa, synthetic construct
  REGION 1..112: note = hu50L1
DIVMTQSPLSLPVTPGEPASISCRSSQSILHSNGNTYLEWYLQKPGQSPQLLIYRVSNRFSGVPDRFSGSGSGTDFTLKISRVEAEDVGVYYCFQGLHVPPTFGQGTKLEIK

SEQ ID NO: 151 - protein, 112 aa, synthetic construct
  REGION 1..112: note = hu50L2
DVFMTQSPLSLPVTPGEPASISCRSSQSILHSNGNTYLEWYLQKPGQSPQLLIYRVSNRFSGVPDRFSGSGSGTDFTLKISRVEAEDVGVYYCFQGLHVPPTFGQGTKLEIK

SEQ ID NO: 152 - protein, 112 aa, synthetic construct
  REGION 1..112: note = hu50L3
DIVMTQSPLSLPVTPGEPASISCRSSQSILHSYGNTYLEWYLQKPGQSPQLLIYRVSNRFSGVPDRFSGSGSGTDFTLKISRVEAEDVGVYYCFQGLHVPPTFGQGTKLEIK

SEQ ID NO: 153 - protein, 119 aa, synthetic construct
  REGION 1..119: note = hu71H1
EVQLVESGGGVVQPGRSLRLSCAASGFTFSNYRMHWVRQAPGKGLEWVAVITVKSDNYGSSYAESVKGRFAISRDNSKNTLYLQMNSLRAEDTAVYYCSRELGQVLVFWGQGTLVTVSS

SEQ ID NO: 154 - protein, 119 aa, synthetic construct
  REGION 1..119: note = hu71H2
EVQLVESGGGVVQPGRSLRLSCATSGFTFSNYRMHWLRQAPGKGLEWVAVITVKSDNYGSSYAESVKGRFAISRDNSKNTLYLQMNSLRAEDTAVYYCSRELGQVLVFWGQGTLVTVSS

SEQ ID NO: 155 - protein, 119 aa, synthetic construct
  REGION 1..119: note = hu71H3
EVQLVESGGGVVQPGRSLRLSCATSGFTFSNYRMHWVRQAPGKGLEWVAVITVKSDNYGSSYAESVKGRFAISREDSKSTLYLQMNSLRAEDTAVYYCSRELGQVLVFWGQGTLVTVSS

SEQ ID NO: 156 - protein, 119 aa, synthetic construct
  REGION 1..119: note = hu71H4
EVQLVESGGGVVQPGRSLRLSCATSGFTFSNYRMHWLRQAPGKRLEWVAVITVKSDNYGSSYAESVKGRFAISREDSKSTLYLQMNSLRAEDTAVYYCSRELGQVLVFWGQGTLVTVSS

SEQ ID NO: 157 - protein, 112 aa, synthetic construct
  REGION 1..112: note = hu71L1
DIVMTQTPLSLPVTPGEPASISCRSSQSLVHSYGNTYLHWYLQKPGQSPQLLIYKVSNRFSGVPDRFSGSGSGTDFTLKISRVEAEDVGVYYCSQTTHVPWTFGGGTKVEIK

SEQ ID NO: 158 - protein, 112 aa, synthetic construct
  REGION 1..112: note = hu71L2
DVVVTQTPLSLPVTPGEPASISCRSSQSLVHSYGNTYLHWYLQKPGQSPQLLIYKVSNRFSGVPDRFSGSGSGTDFTLKISRVEAEDVGVYYCSQTTHVPWTFGGGTKVEIK

SEQ ID NO: 159 - protein, 16 aa, synthetic construct
  REGION 1..16: note = hu50L3 LCDR1
RSSQSILHSYGNTYLE

SEQ ID NO: 160 - protein, 5 aa, synthetic construct
  REGION 1..5: note = S107E HCDR1
KYAMN

SEQ ID NO: 161 - protein, 19 aa, synthetic construct
  REGION 1..19: note = S107E HCDR2
RIRSKYNNYATYYADSVKD

SEQ ID NO: 162 - protein, 14 aa, synthetic construct
  REGION 1..14: note = S107E HCDR3
HGNFGNEYISYWAY

SEQ ID NO: 163 - protein, 14 aa, synthetic construct
  REGION 1..14: note = S107E LCDR1
GSSTGAVTSGNYPN

SEQ ID NO: 164 - protein, 7 aa, synthetic construct
  REGION 1..7: note = S107E LCDR2
GTKFLAP

SEQ ID NO: 165 - protein, 9 aa, synthetic construct
  REGION 1..9: note = S107E LCDR3
VLWYSNRWV

SEQ ID NO: 166 - protein, 125 aa, synthetic construct
  REGION 1..125: note = S107E-VH
EVQLVESGGGLVQPGGSLKLSCAASGFTFNKYAMNWVRQAPGKGLEWVARIRSKYNNYATYYADSVKDRFTISRDDSKNTAYLQMNNLKTEDTAVYYCVRHGNFGNEYISYWAYWGQGTLVTVSS

SEQ ID NO: 167 - protein, 109 aa, synthetic construct
  REGION 1..109: note = S107E-VL
QTVVTQEPSLTVSPGGTVTLTCGSSTGAVTSGNYPNWVQQKPGQAPRGLIGGTKFLAPGTPARFSGSLLGGKAALTLSGVQPEDEAEYYCVLWYSNRWVFGGGTKLTVL

SEQ ID NO: 168 - protein, 103 aa, synthetic construct
  REGION 1..103: note = IgG1(CH1)
ASTKGPSVFPLAPSSKSTSGGTAALGCLVKDYFPEPVTVSWNSGALTSGVHTFPAVLQSSGLYSLSSVVTVPSSSLGTQTYICNVNHKPSNTKVDKKVEPKSC

SEQ ID NO: 169 - protein, 227 aa, synthetic construct
  REGION 1..227: note = IgG1Fc(Knob, L234A/L235A/S354C/T366W)
DKTHTCPPCPAPEAAGGPSVFLFPPKPKDTLMISRTPEVTCVVVDVSHEDPEVKFNWYVDGVEVHNAKTKPREEQYNSTYRVVSVLTVLHQDWLNGKEYKCKVSNKALPAPIEKTISKAKGQPREPQVYTLPPCRDELTKNQVSLWCLVKGFYPSDIAVEWESNGQPENNYKTTPPVLDSDGSFFLYSKLTVDKSRWQQGNVFSCSVMHEALHNHYTQKSLSLSPGK

SEQ ID NO: 170 - protein, 227 aa, synthetic construct
  REGION 1..227: note = IgG1Fc(Hole, L234A/L235A/Y349C/T366S/L368A/Y407Y)
DKTHTCPPCPAPEAAGGPSVFLFPPKPKDTLMISRTPEVTCVVVDVSHEDPEVKFNWYVDGVEVHNAKTKPREEQYNSTYRVVSVLTVLHQDWLNGKEYKCKVSNKALPAPIEKTISKAKGQPREPQVCTLPPSRDELTKNQVSLSCAVKGFYPSDIAVEWESNGQPENNYKTTPPVLDSDGSFFLVSKLTVDKSRWQQGNVFSCSVMHEALHNHYTQKSLSLSPGK

SEQ ID NO: 171 - protein, 454 aa, synthetic construct
  REGION 1..454: note = Ob-hole
EVQLVESGGGLVQPGGSLKLSCAASGFTFNKYAMNWVRQAPGKGLEWVARIRSKYNNYATYYADSVKDRFTISRDDSKNTAYLQMNNLKTEDTAVYYCVRHGNFGNEYISYWAYWGQGTLVTVSSGGGGSSGAPRFLTRPKASVVSVGKDATLSCQIVGNPFPQVSWEKDKQPVTAGVRFRLAQDGDLYRLKILDLQLSDSGQYVCRARNAHGEAFACLGLQVDAEADKTHTCPPCPAPEAAGGPSVFLFPPKPKDTLMISRTPEVTCVVVDVSHEDPEVKFNWYVDGVEVHNAKTKPREEQYNSTYRVVSVLTVLHQDWLNGKEYKCKVSNKALPAPIEKTISKAKGQPREPQVCTLPPSRDELTKNQVSLSCAVKGFYPSDIAVEWESNGQPENNYKTTPPVLDSDGSFFLVSKLTVDKSRWQQGNVFSCSVMHEALHNHYTQKSLSLSPGK

SEQ ID NO: 172 - protein, 212 aa, synthetic construct
  REGION 1..212: note = VL-Titin
QTVVTQEPSLTVSPGGTVTLTCGSSTGAVTSGNYPNWVQQKPGQAPRGLIGGTKFLAPGTPARFSGSLLGGKAALTLSGVQPEDEAEYYCVLWYSNRWVFGGGTKLTVLGGGGSGIPPKIECLPIDISIDEGKVLTVASAFTGEPTPEVTWSTGGRKIHSQEQGRFHIENTDDSTTLTIKDVQKQDGGLYTLTLRNEFGSDSATVNIHIRSI

SEQ ID NO: 173 - protein, 5 aa, synthetic construct
  REGION 1..5: note = linker
GGGGS

SEQ ID NO: 174 - protein, 211 aa, synthetic construct
  REGION 1..211: note = VL-Ob
QTVVTQEPSLTVSPGGTVTLTCGSSTGAVTSGNYPNWVQQKPGQAPRGLIGGTKFLAPGTPARFSGSLLGGKAALTLSGVQPEDEAEYYCVLWYSNRWVFGGGTKLTVLGGGGSSGAPRFLTRPKASVVSVGKDATLSCQIVGNPFPQVSWEKDKQPVTAGVRFRLAQDGDLYRLKILDLQLSDSGQYVCRARNAHGEAFACLGLQVDAEA

SEQ ID NO: 175 - protein, 227 aa, synthetic construct
  REGION 1..227: note = IgG1(AA)Fc
DKTHTCPPCPAPEAAGGPSVFLFPPKPKDTLMISRTPEVTCVVVDVSHEDPEVKFNWYVDGVEVHNAKTKPREEQYNSTYRVVSVLTVLHQDWLNGKEYKCKVSNKALPAPIEKTISKAKGQPREPQVYTLPPSRDELTKNQVSLTCLVKGFYPSDIAVEWESNGQPENNYKTTPPVLDSDGSFFLYSKLTVDKSRWQQGNVFSCSVMHEALHNHYTQKSLSLSPGK

SEQ ID NO: 176 - protein, 15 aa, synthetic construct
  REGION 1..15: note = linker2
GGGGSGGGGSGGGGS

SEQ ID NO: 177 - protein, 12 aa, synthetic construct
  REGION 1..12: note = linker3
GGGTKLTVLGGG

SEQ ID NO: 178 - protein, 6 aa, synthetic construct
  REGION 1..6: note = linker4
SGGGGS

SEQ ID NO: 179 - protein, 4 aa, synthetic construct
  REGION 1..4: note = linker
GGGG

SEQ ID NO: 180 - protein, 450 aa, synthetic construct
  REGION 1..450: note = hu2H1-F2-1
EVQLVESGGGLVQPGGSLRLSCAASGFTFSDYYMAWVRQAPGKGLEWVANINFDGSSTYYLDSLKSRFTISRDNAKNSLYLQMNSLRAEDTAVYYCARDLDGYYGYFDVWGQGTTVTVSSASTKGPSVFPLAPSSKSTSGGTAALGCLVKDYFPEPVTVSWNSGALTSGVHTFPAVLQSSGLYSLSSVVTVPSSSLGTQTYICNVNHKPSNTKVDKKVEPKSCDKTHTCPPCPAPEAAGGPSVFLFPPKPKDTLMISRTPEVTCVVVDVSHEDPEVKFNWYVDGVEVHNAKTKPREEQYNSTYRVVSVLTVLHQDWLNGKEYKCKVSNKALPAPIEKTISKAKGQPREPQVYTLPPCRDELTKNQVSLWCLVKGFYPSDIAVEWESNGQPENNYKTTPPVLDSDGSFFLYSKLTVDKSRWQQGNVFSCSVMHEALHNHYTQKSLSLSPGK

SEQ ID NO: 181 - protein, 213 aa, synthetic construct
  REGION 1..213: note = hu2L1-CL
EIVLTQSPDFQSVTPKEKVTITCSASSSVSHMYWYQQKPDQSPKLLIYRTSNLASGVPSRFSGSGSGTDFTLTINSLEAEDAATYYCQQYHSYPLMFGQGTKLEIKRTVAAPSVFIFPPSDEQLKSGTASVVCLLNNFYPREAKVQWKVDNALQSGNSQESVTEQDSKDSTYSLSSTLTLSKADYEKHKVYACEVTHQGLSSPVTKSFNRGEC

SEQ ID NO: 182 - protein, 678 aa, synthetic construct
  REGION 1..678: note = hu2H1-F2-3
EVQLVESGGGLVQPGGSLRLSCAASGFTFSDYYMAWVRQAPGKGLEWVANINFDGSSTYYLDSLKSRFTISRDNAKNSLYLQMNSLRAEDTAVYYCARDLDGYYGYFDVWGQGTTVTVSSASTKGPSVFPLAPSSKSTSGGTAALGCLVKDYFPEPVTVSWNSGALTSGVHTFPAVLQSSGLYSLSSVVTVPSSSLGTQTYICNVNHKPSNTKVDKKVEPKSCEVQLVESGGGLVQPGGSLKLSCAASGFTFNKYAMNWVRQAPGKGLEWVARIRSKYNNYATYYADSVKDRFTISRDDSKNTAYLQMNNLKTEDTAVYYCVRHGNFGNEYISYWAYWGQGTLVTVSSGGGGSGIPPKIECLPIDISIDEGKVLTVASAFTGEPTPEVTWSTGGRKIHSQEQGRFHIENTDDSTTLTIKDVQKQDGGLYTLTLRNEFGSDSATVNIHIRSIDKTHTCPPCPAPEAAGGPSVFLFPPKPKDTLMISRTPEVTCVVVDVSHEDPEVKFNWYVDGVEVHNAKTKPREEQYNSTYRVVSVLTVLHQDWLNGKEYKCKVSNKALPAPIEKTISKAKGQPREPQVCTLPPSRDELTKNQVSLSCAVKGFYPSDIAVEWESNGQPENNYKTTPPVLDSDGSFFLVSKLTVDKSRWQQGNVFSCSVMHEALHNHYTQKSLSLSPGK

SEQ ID NO: 183 - protein, 678 aa, synthetic construct
  REGION 1..678: note = hu2H1-F3-1
EVQLVESGGGLVQPGGSLRLSCAASGFTFSDYYMAWVRQAPGKGLEWVANINFDGSSTYYLDSLKSRFTISRDNAKNSLYLQMNSLRAEDTAVYYCARDLDGYYGYFDVWGQGTTVTVSSASTKGPSVFPLAPSSKSTSGGTAALGCLVKDYFPEPVTVSWNSGALTSGVHTFPAVLQSSGLYSLSSVVTVPSSSLGTQTYICNVNHKPSNTKVDKKVEPKSCEVQLVESGGGLVQPGGSLKLSCAASGFTFNKYAMNWVRQAPGKGLEWVARIRSKYNNYATYYADSVKDRFTISRDDSKNTAYLQMNNLKTEDTAVYYCVRHGNFGNEYISYWAYWGQGTLVTVSSGGGGSGIPPKIECLPIDISIDEGKVLTVASAFTGEPTPEVTWSTGGRKIHSQEQGRFHIENTDDSTTLTIKDVQKQDGGLYTLTLRNEFGSDSATVNIHIRSIDKTHTCPPCPAPEAAGGPSVFLFPPKPKDTLMISRTPEVTCVVVDVSHEDPEVKFNWYVDGVEVHNAKTKPREEQYNSTYRVVSVLTVLHQDWLNGKEYKCKVSNKALPAPIEKTISKAKGQPREPQVYTLPPSRDELTKNQVSLTCLVKGFYPSDIAVEWESNGQPENNYKTTPPVLDSDGSFFLYSKLTVDKSRWQQGNVFSCSVMHEALHNHYTQKSLSLSPGK

SEQ ID NO: 184 - protein, 702 aa, synthetic construct
  REGION 1..702: note = hu2H1-F4-1
EVQLVESGGGLVQPGGSLRLSCAASGFTFSDYYMAWVRQAPGKGLEWVANINFDGSSTYYLDSLKSRFTISRDNAKNSLYLQMNSLRAEDTAVYYCARDLDGYYGYFDVWGQGTTVTVSSASTKGPSVFPLAPSSKSTSGGTAALGCLVKDYFPEPVTVSWNSGALTSGVHTFPAVLQSSGLYSLSSVVTVPSSSLGTQTYICNVNHKPSNTKVDKKVEPKSCEVQLVESGGGLVQPGGSLKLSCAASGFTFNKYAMNWVRQAPGKGLEWVARIRSKYNNYATYYADSVKDRFTISRDDSKNTAYLQMNNLKTEDTAVYYCVRHGNFGNEYISYWAYWGQGTLVTVSSGGGGSGGGGSGGGGSQTVVTQEPSLTVSPGGTVTLTCGSSTGAVTSGNYPNWVQQKPGQAPRGLIGGTKFLAPGTPARFSGSLLGGKAALTLSGVQPEDEAEYYCVLWYSNRWVFGGGTKLTVLGGGDKTHTCPPCPAPEAAGGPSVFLFPPKPKDTLMISRTPEVTCVVVDVSHEDPEVKFNWYVDGVEVHNAKTKPREEQYNSTYRVVSVLTVLHQDWLNGKEYKCKVSNKALPAPIEKTISKAKGQPREPQVYTLPPSRDELTKNQVSLTCLVKGFYPSDIAVEWESNGQPENNYKTTPPVLDSDGSFFLYSKLTVDKSRWQQGNVFSCSVMHEALHNHYTQKSLSLSPGK

SEQ ID NO: 185 - protein, 682 aa, synthetic construct
  REGION 1..682: note = hu13H1-F3-1
EVTLKESGPVLVKPTETLTLTCTVSGFSLSNYAISWIRQPPGKALEWLAVIWTGGGTHYNSALKSRLTISKDTSKSQVVLTMTNMDPVDTATYYCARKGNYYGSSLYYYAMNYWGQGTTVTVSSASTKGPSVFPLAPSSKSTSGGTAALGCLVKDYFPEPVTVSWNSGALTSGVHTFPAVLQSSGLYSLSSVVTVPSSSLGTQTYICNVNHKPSNTKVDKKVEPKSCEVQLVESGGGLVQPGGSLKLSCAASGFTFNKYAMNWVRQAPGKGLEWVARIRSKYNNYATYYADSVKDRFTISRDDSKNTAYLQMNNLKTEDTAVYYCVRHGNFGNEYISYWAYWGQGTLVTVSSGGGGSGIPPKIECLPIDISIDEGKVLTVASAFTGEPTPEVTWSTGGRKIHSQEQGRFHIENTDDSTTLTIKDVQKQDGGLYTLTLRNEFGSDSATVNIHIRSIDKTHTCPPCPAPEAAGGPSVFLFPPKPKDTLMISRTPEVTCVVVDVSHEDPEVKFNWYVDGVEVHNAKTKPREEQYNSTYRVVSVLTVLHQDWLNGKEYKCKVSNKALPAPIEKTISKAKGQPREPQVYTLPPSRDELTKNQVSLTCLVKGFYPSDIAVEWESNGQPENNYKTTPPVLDSDGSFFLYSKLTVDKSRWQQGNVFSCSVMHEALHNHYTQKSLSLSPGK

SEQ ID NO: 186 - protein, 214 aa, synthetic construct
  REGION 1..214: note = hu13L1-CL
DIQMTQSPSSLSASVGDRVTITCRASQDISNYLNWYQQKPGKAPKLLIYYTSRLQSGVPSRFSGSGSGTDFTLTISSLQPEDFATYYCQQGDTLPYTFGGGTKVEIKRTVAAPSVFIFPPSDEQLKSGTASVVCLLNNFYPREAKVQWKVDNALQSGNSQESVTEQDSKDSTYSLSSTLTLSKADYEKHKVYACEVTHQGLSSPVTKSFNRGEC

SEQ ID NO: 187 - protein, 446 aa, synthetic construct
  REGION 1..446: note = hu15H4-F2-1
EFQLVQSGAEVKKPGASVKVSCKASGYSFTDHNMNWVRQAPGQRLEWMGLINPNYGTADYNQKFKGRVTLTVDQSATTAYMELSSLRSEDTAVYYCARGSSLFAYWGQGTLVTVSSASTKGPSVFPLAPSSKSTSGGTAALGCLVKDYFPEPVTVSWNSGALTSGVHTFPAVLQSSGLYSLSSVVTVPSSSLGTQTYICNVNHKPSNTKVDKKVEPKSCDKTHTCPPCPAPEAAGGPSVFLFPPKPKDTLMISRTPEVTCVVVDVSHEDPEVKFNWYVDGVEVHNAKTKPREEQYNSTYRVVSVLTVLHQDWLNGKEYKCKVSNKALPAPIEKTISKAKGQPREPQVYTLPPCRDELTKNQVSLWCLVKGFYPSDIAVEWESNGQPENNYKTTPPVLDSDGSFFLYSKLTVDKSRWQQGNVFSCSVMHEALHNHYTQKSLSLSPGK

SEQ ID NO: 188 - protein, 214 aa, synthetic construct
  REGION 1..214: note = hu15L2-CL
DIQMTQSPSSLSASVGDRVTITCKASQGVDTAVAWYQQKPGKSPKLLIYWASTRHTGVPDRFSGSGSGTDFTLTISSLQPEDVATYYCQQYSRYPLTFGQGTKLEIKRTVAAPSVFIFPPSDEQLKSGTASVVCLLNNFYPREAKVQWKVDNALQSGNSQESVTEQDSKDSTYSLSSTLTLSKADYEKHKVYACEVTHQGLSSPVTKSFNRGEC

SEQ ID NO: 189 - protein, 674 aa, synthetic construct
  REGION 1..674: note = hu15H4-F2-3
EFQLVQSGAEVKKPGASVKVSCKASGYSFTDHNMNWVRQAPGQRLEWMGLINPNYGTADYNQKFKGRVTLTVDQSATTAYMELSSLRSEDTAVYYCARGSSLFAYWGQGTLVTVSSASTKGPSVFPLAPSSKSTSGGTAALGCLVKDYFPEPVTVSWNSGALTSGVHTFPAVLQSSGLYSLSSVVTVPSSSLGTQTYICNVNHKPSNTKVDKKVEPKSCEVQLVESGGGLVQPGGSLKLSCAASGFTFNKYAMNWVRQAPGKGLEWVARIRSKYNNYATYYADSVKDRFTISRDDSKNTAYLQMNNLKTEDTAVYYCVRHGNFGNEYISYWAYWGQGTLVTVSSGGGGSGIPPKIECLPIDISIDEGKVLTVASAFTGEPTPEVTWSTGGRKIHSQEQGRFHIENTDDSTTLTIKDVQKQDGGLYTLTLRNEFGSDSATVNIHIRSIDKTHTCPPCPAPEAAGGPSVFLFPPKPKDTLMISRTPEVTCVVVDVSHEDPEVKFNWYVDGVEVHNAKTKPREEQYNSTYRVVSVLTVLHQDWLNGKEYKCKVSNKALPAPIEKTISKAKGQPREPQVCTLPPSRDELTKNQVSLSCAVKGFYPSDIAVEWESNGQPENNYKTTPPVLDSDGSFFLVSKLTVDKSRWQQGNVFSCSVMHEALHNHYTQKSLSLSPGK

SEQ ID NO: 190 - protein, 698 aa, synthetic construct
  REGION 1..698: note = hu15H4-F4-1
EFQLVQSGAEVKKPGASVKVSCKASGYSFTDHNMNWVRQAPGQRLEWMGLINPNYGTADYNQKFKGRVTLTVDQSATTAYMELSSLRSEDTAVYYCARGSSLFAYWGQGTLVTVSSASTKGPSVFPLAPSSKSTSGGTAALGCLVKDYFPEPVTVSWNSGALTSGVHTFPAVLQSSGLYSLSSVVTVPSSSLGTQTYICNVNHKPSNTKVDKKVEPKSCEVQLVESGGGLVQPGGSLKLSCAASGFTFNKYAMNWVRQAPGKGLEWVARIRSKYNNYATYYADSVKDRFTISRDDSKNTAYLQMNNLKTEDTAVYYCVRHGNFGNEYISYWAYWGQGTLVTVSSGGGGSGGGGSGGGGSQTVVTQEPSLTVSPGGTVTLTCGSSTGAVTSGNYPNWVQQKPGQAPRGLIGGTKFLAPGTPARFSGSLLGGKAALTLSGVQPEDEAEYYCVLWYSNRWVFGGGTKLTVLGGGDKTHTCPPCPAPEAAGGPSVFLFPPKPKDTLMISRTPEVTCVVVDVSHEDPEVKFNWYVDGVEVHNAKTKPREEQYNSTYRVVSVLTVLHQDWLNGKEYKCKVSNKALPAPIEKTISKAKGQPREPQVYTLPPSRDELTKNQVSLTCLVKGFYPSDIAVEWESNGQPENNYKTTPPVLDSDGSFFLYSKLTVDKSRWQQGNVFSCSVMHEALHNHYTQKSLSLSPGK

SEQ ID NO: 191 - protein, 723 aa, synthetic construct
  REGION 1..723: note = hu15H4L2-F5-1
EFQLVQSGAEVKKPGASVKVSCKASGYSFTDHNMNWVRQAPGQRLEWMGLINPNYGTADYNQKFKGRVTLTVDQSATTAYMELSSLRSEDTAVYYCARGSSLFAYWGQGTLVTVSSGGGGSGGGGSGGGGSDIQMTQSPSSLSASVGDRVTITCKASQGVDTAVAWYQQKPGKSPKLLIYWASTRHTGVPDRFSGSGSGTDFTLTISSLQPEDVATYYCQQYSRYPLTFGQGTKLEIKSGGGGSEVQLVESGGGLVQPGGSLKLSCAASGFTFNKYAMNWVRQAPGKGLEWVARIRSKYNNYATYYADSVKDRFTISRDDSKNTAYLQMNNLKTEDTAVYYCVRHGNFGNEYISYWAYWGQGTLVTVSSGGGGSGGGGSGGGGSQTVVTQEPSLTVSPGGTVTLTCGSSTGAVTSGNYPNWVQQKPGQAPRGLIGGTKFLAPGTPARFSGSLLGGKAALTLSGVQPEDEAEYYCVLWYSNRWVFGGGTKLTVLGGGDKTHTCPPCPAPEAAGGPSVFLFPPKPKDTLMISRTPEVTCVVVDVSHEDPEVKFNWYVDGVEVHNAKTKPREEQYNSTYRVVSVLTVLHQDWLNGKEYKCKVSNKALPAPIEKTISKAKGQPREPQVCTLPPSRDELTKNQVSLSCAVKGFYPSDIAVEWESNGQPENNYKTTPPVLDSDGSFFLVSKLTVDKSRWQQGNVFSCSVMHEALHNHYTQKSLSLSPGK

SEQ ID NO: 192 - protein, 723 aa, synthetic construct
  REGION 1..723: note = hu15H6L3-F5-1
EFQLVQSGAEVKKPGASVKVSCKASGYSFTDHNMNWVRQAPGQCLEWMGLINPNYGTADYNQKFKGRVTLTVDQSATTAYMELSSLRSEDTAVYYCARGSSLFAYWGQGTLVTVSSGGGGSGGGGSGGGGSDIQMTQSPSSLSASVGDRVTITCKASQGVDTAVAWYQQKPGKSPKLLIYWASTRHTGVPDRFSGSGSGTDFTLTISSLQPEDVATYYCQQYSRYPLTFGCGTKLEIKSGGGGSEVQLVESGGGLVQPGGSLKLSCAASGFTFNKYAMNWVRQAPGKGLEWVARIRSKYNNYATYYADSVKDRFTISRDDSKNTAYLQMNNLKTEDTAVYYCVRHGNFGNEYISYWAYWGQGTLVTVSSGGGGSGGGGSGGGGSQTVVTQEPSLTVSPGGTVTLTCGSSTGAVTSGNYPNWVQQKPGQAPRGLIGGTKFLAPGTPARFSGSLLGGKAALTLSGVQPEDEAEYYCVLWYSNRWVFGGGTKLTVLGGGDKTHTCPPCPAPEAAGGPSVFLFPPKPKDTLMISRTPEVTCVVVDVSHEDPEVKFNWYVDGVEVHNAKTKPREEQYNSTYRVVSVLTVLHQDWLNGKEYKCKVSNKALPAPIEKTISKAKGQPREPQVCTLPPSRDELTKNQVSLSCAVKGFYPSDIAVEWESNGQPENNYKTTPPVLDSDGSFFLVSKLTVDKSRWQQGNVFSCSVMHEALHNHYTQKSLSLSPGK

SEQ ID NO: 193 - protein, 449 aa, synthetic construct
  REGION 1..449: note = hu19H2-F1-1
EVKLVESGGGLVQPGGSLRLSCAASGFTFSDYYMAWVRQAPGKGLEWVANINYDGSSTYYLDSLKSRFTISRDNAKNSLYLQMNSLRAEDTAVYYCARGGDYWDAMDYWGQGTTVTVSSASTKGPSVFPLAPSSKSTSGGTAALGCLVKDYFPEPVTVSWNSGALTSGVHTFPAVLQSSGLYSLSSVVTVPSSSLGTQTYICNVNHKPSNTKVDKKVEPKSCDKTHTCPPCPAPEAAGGPSVFLFPPKPKDTLMISRTPEVTCVVVDVSHEDPEVKFNWYVDGVEVHNAKTKPREEQYNSTYRVVSVLTVLHQDWLNGKEYKCKVSNKALPAPIEKTISKAKGQPREPQVYTLPPCRDELTKNQVSLWCLVKGFYPSDIAVEWESNGQPENNYKTTPPVLDSDGSFFLYSKLTVDKSRWQQGNVFSCSVMHEALHNHYTQKSLSLSPGK

SEQ ID NO: 194 - protein, 214 aa, synthetic construct
  REGION 1..214: note = hu19L2-CL
DIQMTQSPSSLSASVGDRVTITCRASQDISKYLNWYQQKPGKAPKLLIYYTSSLHSGVPSRFSGSGSGTDYTLTISSLQPEDFATYYCQQGNRLPRTFGGGTKVEIKRTVAAPSVFIFPPSDEQLKSGTASVVCLLNNFYPREAKVQWKVDNALQSGNSQESVTEQDSKDSTYSLSSTLTLSKADYEKHKVYACEVTHQGLSSPVTKSFNRGEC

SEQ ID NO: 195 - protein, 677 aa, synthetic construct
  REGION 1..677: note = hu19H2-F2-3
EVKLVESGGGLVQPGGSLRLSCAASGFTFSDYYMAWVRQAPGKGLEWVANINYDGSSTYYLDSLKSRFTISRDNAKNSLYLQMNSLRAEDTAVYYCARGGDYWDAMDYWGQGTTVTVSSASTKGPSVFPLAPSSKSTSGGTAALGCLVKDYFPEPVTVSWNSGALTSGVHTFPAVLQSSGLYSLSSVVTVPSSSLGTQTYICNVNHKPSNTKVDKKVEPKSCEVQLVESGGGLVQPGGSLKLSCAASGFTFNKYAMNWVRQAPGKGLEWVARIRSKYNNYATYYADSVKDRFTISRDDSKNTAYLQMNNLKTEDTAVYYCVRHGNFGNEYISYWAYWGQGTLVTVSSGGGGSGIPPKIECLPIDISIDEGKVLTVASAFTGEPTPEVTWSTGGRKIHSQEQGRFHIENTDDSTTLTIKDVQKQDGGLYTLTLRNEFGSDSATVNIHIRSIDKTHTCPPCPAPEAAGGPSVFLFPPKPKDTLMISRTPEVTCVVVDVSHEDPEVKFNWYVDGVEVHNAKTKPREEQYNSTYRVVSVLTVLHQDWLNGKEYKCKVSNKALPAPIEKTISKAKGQPREPQVCTLPPSRDELTKNQVSLSCAVKGFYPSDIAVEWESNGQPENNYKTTPPVLDSDGSFFLVSKLTVDKSRWQQGNVFSCSVMHEALHNHYTQKSLSLSPGK

SEQ ID NO: 196 - protein, 677 aa, synthetic construct
  REGION 1..677: note = hu19H2-F3-1
EVKLVESGGGLVQPGGSLRLSCAASGFTFSDYYMAWVRQAPGKGLEWVANINYDGSSTYYLDSLKSRFTISRDNAKNSLYLQMNSLRAEDTAVYYCARGGDYWDAMDYWGQGTTVTVSSASTKGPSVFPLAPSSKSTSGGTAALGCLVKDYFPEPVTVSWNSGALTSGVHTFPAVLQSSGLYSLSSVVTVPSSSLGTQTYICNVNHKPSNTKVDKKVEPKSCEVQLVESGGGLVQPGGSLKLSCAASGFTFNKYAMNWVRQAPGKGLEWVARIRSKYNNYATYYADSVKDRFTISRDDSKNTAYLQMNNLKTEDTAVYYCVRHGNFGNEYISYWAYWGQGTLVTVSSGGGGSGIPPKIECLPIDISIDEGKVLTVASAFTGEPTPEVTWSTGGRKIHSQEQGRFHIENTDDSTTLTIKDVQKQDGGLYTLTLRNEFGSDSATVNIHIRSIDKTHTCPPCPAPEAAGGPSVFLFPPKPKDTLMISRTPEVTCVVVDVSHEDPEVKFNWYVDGVEVHNAKTKPREEQYNSTYRVVSVLTVLHQDWLNGKEYKCKVSNKALPAPIEKTISKAKGQPREPQVYTLPPSRDELTKNQVSLTCLVKGFYPSDIAVEWESNGQPENNYKTTPPVLDSDGSFFLYSKLTVDKSRWQQGNVFSCSVMHEALHNHYTQKSLSLSPGK

SEQ ID NO: 197 - protein, 701 aa, synthetic construct
  REGION 1..701: note = hu19H2-F4-1
EVKLVESGGGLVQPGGSLRLSCAASGFTFSDYYMAWVRQAPGKGLEWVANINYDGSSTYYLDSLKSRFTISRDNAKNSLYLQMNSLRAEDTAVYYCARGGDYWDAMDYWGQGTTVTVSSASTKGPSVFPLAPSSKSTSGGTAALGCLVKDYFPEPVTVSWNSGALTSGVHTFPAVLQSSGLYSLSSVVTVPSSSLGTQTYICNVNHKPSNTKVDKKVEPKSCEVQLVESGGGLVQPGGSLKLSCAASGFTFNKYAMNWVRQAPGKGLEWVARIRSKYNNYATYYADSVKDRFTISRDDSKNTAYLQMNNLKTEDTAVYYCVRHGNFGNEYISYWAYWGQGTLVTVSSGGGGSGGGGSGGGGSQTVVTQEPSLTVSPGGTVTLTCGSSTGAVTSGNYPNWVQQKPGQAPRGLIGGTKFLAPGTPARFSGSLLGGKAALTLSGVQPEDEAEYYCVLWYSNRWVFGGGTKLTVLGGGDKTHTCPPCPAPEAAGGPSVFLFPPKPKDTLMISRTPEVTCVVVDVSHEDPEVKFNWYVDGVEVHNAKTKPREEQYNSTYRVVSVLTVLHQDWLNGKEYKCKVSNKALPAPIEKTISKAKGQPREPQVYTLPPSRDELTKNQVSLTCLVKGFYPSDIAVEWESNGQPENNYKTTPPVLDSDGSFFLYSKLTVDKSRWQQGNVFSCSVMHEALHNHYTQKSLSLSPGK

SEQ ID NO: 198 - protein, 726 aa, synthetic construct
  REGION 1..726: note = hu19H2-F5-1
EVKLVESGGGLVQPGGSLRLSCAASGFTFSDYYMAWVRQAPGKGLEWVANINYDGSSTYYLDSLKSRFTISRDNAKNSLYLQMNSLRAEDTAVYYCARGGDYWDAMDYWGQGTTVTVSSGGGGSGGGGSGGGGSDIQMTQSPSSLSASVGDRVTITCRASQDISKYLNWYQQKPGKAPKLLIYYTSSLHSGVPSRFSGSGSGTDYTLTISSLQPEDFATYYCQQGNRLPRTFGGGTKVEIKSGGGGSEVQLVESGGGLVQPGGSLKLSCAASGFTFNKYAMNWVRQAPGKGLEWVARIRSKYNNYATYYADSVKDRFTISRDDSKNTAYLQMNNLKTEDTAVYYCVRHGNFGNEYISYWAYWGQGTLVTVSSGGGGSGGGGSGGGGSQTVVTQEPSLTVSPGGTVTLTCGSSTGAVTSGNYPNWVQQKPGQAPRGLIGGTKFLAPGTPARFSGSLLGGKAALTLSGVQPEDEAEYYCVLWYSNRWVFGGGTKLTVLGGGDKTHTCPPCPAPEAAGGPSVFLFPPKPKDTLMISRTPEVTCVVVDVSHEDPEVKFNWYVDGVEVHNAKTKPREEQYNSTYRVVSVLTVLHQDWLNGKEYKCKVSNKALPAPIEKTISKAKGQPREPQVCTLPPSRDELTKNQVSLSCAVKGFYPSDIAVEWESNGQPENNYKTTPPVLDSDGSFFLVSKLTVDKSRWQQGNVFSCSVMHEALHNHYTQKSLSLSPGK

SEQ ID NO: 199 - protein, 702 aa, synthetic construct
  REGION 1..702: note = hu27H1-F4-1
EVQLVESGGGLVQPGGSLRLSCAASGFTFSDYYMAWVRQAPGKGLEWVANINYDGSSTYYLDSLKSRFTISRDNAKNSLYLQMNSLRAEDTAVYYCARDLDGYYGYFDVWGQGTTVTVSSASTKGPSVFPLAPSSKSTSGGTAALGCLVKDYFPEPVTVSWNSGALTSGVHTFPAVLQSSGLYSLSSVVTVPSSSLGTQTYICNVNHKPSNTKVDKKVEPKSCEVQLVESGGGLVQPGGSLKLSCAASGFTFNKYAMNWVRQAPGKGLEWVARIRSKYNNYATYYADSVKDRFTISRDDSKNTAYLQMNNLKTEDTAVYYCVRHGNFGNEYISYWAYWGQGTLVTVSSGGGGSGGGGSGGGGSQTVVTQEPSLTVSPGGTVTLTCGSSTGAVTSGNYPNWVQQKPGQAPRGLIGGTKFLAPGTPARFSGSLLGGKAALTLSGVQPEDEAEYYCVLWYSNRWVFGGGTKLTVLGGGDKTHTCPPCPAPEAAGGPSVFLFPPKPKDTLMISRTPEVTCVVVDVSHEDPEVKFNWYVDGVEVHNAKTKPREEQYNSTYRVVSVLTVLHQDWLNGKEYKCKVSNKALPAPIEKTISKAKGQPREPQVYTLPPSRDELTKNQVSLTCLVKGFYPSDIAVEWESNGQPENNYKTTPPVLDSDGSFFLYSKLTVDKSRWQQGNVFSCSVMHEALHNHYTQKSLSLSPGK

SEQ ID NO: 200 - protein, 213 aa, synthetic construct
  REGION 1..213: note = hu27L6-CL
QIVLTQSPDFQSVTPKEKVTIQCSASSSVSYMYWYQQKPDQSPKPWIYRTSNLASGVPSRFSGSGSGTDYTLTINSLEAEDAATYYCQQYHSYPLTFGQGTKLEIKRTVAAPSVFIFPPSDEQLKSGTASVVCLLNNFYPREAKVQWKVDNALQSGNSQESVTEQDSKDSTYSLSSTLTLSKADYEKHKVYACEVTHQGLSSPVTKSFNRGEC

SEQ ID NO: 201 - protein, 449 aa, synthetic construct
  REGION 1..449: note = hu31H1-F1-1
EVQLVESGGGLVQPGGSLRLSCAASGFTFSDYYMAWVRQAPGKGLEWVASINYDGSSTYYLDSLKSRFTISRDNAKNSLYLQMNSLRAEDTAVYYCAGSDGYWAWFAYWGQGTLVTVSSASTKGPSVFPLAPSSKSTSGGTAALGCLVKDYFPEPVTVSWNSGALTSGVHTFPAVLQSSGLYSLSSVVTVPSSSLGTQTYICNVNHKPSNTKVDKKVEPKSCDKTHTCPPCPAPEAAGGPSVFLFPPKPKDTLMISRTPEVTCVVVDVSHEDPEVKFNWYVDGVEVHNAKTKPREEQYNSTYRVVSVLTVLHQDWLNGKEYKCKVSNKALPAPIEKTISKAKGQPREPQVYTLPPCRDELTKNQVSLWCLVKGFYPSDIAVEWESNGQPENNYKTTPPVLDSDGSFFLYSKLTVDKSRWQQGNVFSCSVMHEALHNHYTQKSLSLSPGK

SEQ ID NO: 202 - protein, 214 aa, synthetic construct
  REGION 1..214: note = hu31L1-CL
DIQMTQSPSSLSASVGDRVTITCRASGNIHNYLAWYQQKPGKAPKLLIYNAETLADGVPSRFSGSGSGTDFTLTISSLQPEDFATYYCQHFWSTPPTFGGGTKVEIKRTVAAPSVFIFPPSDEQLKSGTASVVCLLNNFYPREAKVQWKVDNALQSGNSQESVTEQDSKDSTYSLSSTLTLSKADYEKHKVYACEVTHQGLSSPVTKSFNRGEC

SEQ ID NO: 203 - protein, 680 aa, synthetic construct
  REGION 1..680: note = hu43H3-F3-1
EVQFVESGGGLVQPGGSLRLSCAASGFTFSNYWMNWLRQAPGKGLEWVAQVRLKSDNYATHYAESVKGRFTISREDAKNSAYLQMNSLRAEDTAVYYCSENYYGPAGPFDFWGQGTTVTVSSASTKGPSVFPLAPSSKSTSGGTAALGCLVKDYFPEPVTVSWNSGALTSGVHTFPAVLQSSGLYSLSSVVTVPSSSLGTQTYICNVNHKPSNTKVDKKVEPKSCEVQLVESGGGLVQPGGSLKLSCAASGFTFNKYAMNWVRQAPGKGLEWVARIRSKYNNYATYYADSVKDRFTISRDDSKNTAYLQMNNLKTEDTAVYYCVRHGNFGNEYISYWAYWGQGTLVTVSSGGGGSGIPPKIECLPIDISIDEGKVLTVASAFTGEPTPEVTWSTGGRKIHSQEQGRFHIENTDDSTTLTIKDVQKQDGGLYTLTLRNEFGSDSATVNIHIRSIDKTHTCPPCPAPEAAGGPSVFLFPPKPKDTLMISRTPEVTCVVVDVSHEDPEVKFNWYVDGVEVHNAKTKPREEQYNSTYRVVSVLTVLHQDWLNGKEYKCKVSNKALPAPIEKTISKAKGQPREPQVYTLPPSRDELTKNQVSLTCLVKGFYPSDIAVEWESNGQPENNYKTTPPVLDSDGSFFLYSKLTVDKSRWQQGNVFSCSVMHEALHNHYTQKSLSLSPGK

SEQ ID NO: 204 - protein, 214 aa, synthetic construct
  REGION 1..214: note = hu43L2-CL
DIQMTQSPSSLSASVGDRVTITCKASQNVHTSVAWYQQKPGKSPKLLIYSASNRYSGVPSRFSGSGSGTDFTLTISSLQPEDVATYYCQQYSSYPLTFGQGTKLEIKRTVAAPSVFIFPPSDEQLKSGTASVVCLLNNFYPREAKVQWKVDNALQSGNSQESVTEQDSKDSTYSLSSTLTLSKADYEKHKVYACEVTHQGLSSPVTKSFNRGEC

SEQ ID NO: 205 - protein, 704 aa, synthetic construct
  REGION 1..704: note = hu43H3-F4-1
EVQFVESGGGLVQPGGSLRLSCAASGFTFSNYWMNWLRQAPGKGLEWVAQVRLKSDNYATHYAESVKGRFTISREDAKNSAYLQMNSLRAEDTAVYYCSENYYGPAGPFDFWGQGTTVTVSSASTKGPSVFPLAPSSKSTSGGTAALGCLVKDYFPEPVTVSWNSGALTSGVHTFPAVLQSSGLYSLSSVVTVPSSSLGTQTYICNVNHKPSNTKVDKKVEPKSCEVQLVESGGGLVQPGGSLKLSCAASGFTFNKYAMNWVRQAPGKGLEWVARIRSKYNNYATYYADSVKDRFTISRDDSKNTAYLQMNNLKTEDTAVYYCVRHGNFGNEYISYWAYWGQGTLVTVSSGGGGSGGGGSGGGGSQTVVTQEPSLTVSPGGTVTLTCGSSTGAVTSGNYPNWVQQKPGQAPRGLIGGTKFLAPGTPARFSGSLLGGKAALTLSGVQPEDEAEYYCVLWYSNRWVFGGGTKLTVLGGGDKTHTCPPCPAPEAAGGPSVFLFPPKPKDTLMISRTPEVTCVVVDVSHEDPEVKFNWYVDGVEVHNAKTKPREEQYNSTYRVVSVLTVLHQDWLNGKEYKCKVSNKALPAPIEKTISKAKGQPREPQVYTLPPSRDELTKNQVSLTCLVKGFYPSDIAVEWESNGQPENNYKTTPPVLDSDGSFFLYSKLTVDKSRWQQGNVFSCSVMHEALHNHYTQKSLSLSPGK

SEQ ID NO: 206 - protein, 445 aa, synthetic construct
  REGION 1..445: note = hu46H2-F2-1
EVQLVESGGGLVKPGGSLRLSCAASGFTFSNYGMSWVRQAPGKGLEWVSTIGSGGGYTYYSDSVKGRFTISRDNAKNSLYLQMNSLRAEDTAVYYCVRHPQIGYWGQGTLVTVSSASTKGPSVFPLAPSSKSTSGGTAALGCLVKDYFPEPVTVSWNSGALTSGVHTFPAVLQSSGLYSLSSVVTVPSSSLGTQTYICNVNHKPSNTKVDKKVEPKSCDKTHTCPPCPAPEAAGGPSVFLFPPKPKDTLMISRTPEVTCVVVDVSHEDPEVKFNWYVDGVEVHNAKTKPREEQYNSTYRVVSVLTVLHQDWLNGKEYKCKVSNKALPAPIEKTISKAKGQPREPQVYTLPPCRDELTKNQVSLWCLVKGFYPSDIAVEWESNGQPENNYKTTPPVLDSDGSFFLYSKLTVDKSRWQQGNVFSCSVMHEALHNHYTQKSLSLSPGK

SEQ ID NO: 207 - protein, 214 aa, synthetic construct
  REGION 1..214: note = hu46L2-CL
DIQMTQSPSSLSASVGDRVTITCKASQSVGTAVAWYQQKPGKAPKLLIYSASSRYTGVPSRFSGSGSGTDFTLTISSLQPEDFADYFCHQYSSYPLTFGGGTKVEIKRTVAAPSVFIFPPSDEQLKSGTASVVCLLNNFYPREAKVQWKVDNALQSGNSQESVTEQDSKDSTYSLSSTLTLSKADYEKHKVYACEVTHQGLSSPVTKSFNRGEC

SEQ ID NO: 208 - protein, 673 aa, synthetic construct
  REGION 1..673: note = hu46H2-F2-3
EVQLVESGGGLVKPGGSLRLSCAASGFTFSNYGMSWVRQAPGKGLEWVSTIGSGGGYTYYSDSVKGRFTISRDNAKNSLYLQMNSLRAEDTAVYYCVRHPQIGYWGQGTLVTVSSASTKGPSVFPLAPSSKSTSGGTAALGCLVKDYFPEPVTVSWNSGALTSGVHTFPAVLQSSGLYSLSSVVTVPSSSLGTQTYICNVNHKPSNTKVDKKVEPKSCEVQLVESGGGLVQPGGSLKLSCAASGFTFNKYAMNWVRQAPGKGLEWVARIRSKYNNYATYYADSVKDRFTISRDDSKNTAYLQMNNLKTEDTAVYYCVRHGNFGNEYISYWAYWGQGTLVTVSSGGGGSGIPPKIECLPIDISIDEGKVLTVASAFTGEPTPEVTWSTGGRKIHSQEQGRFHIENTDDSTTLTIKDVQKQDGGLYTLTLRNEFGSDSATVNIHIRSIDKTHTCPPCPAPEAAGGPSVFLFPPKPKDTLMISRTPEVTCVVVDVSHEDPEVKFNWYVDGVEVHNAKTKPREEQYNSTYRVVSVLTVLHQDWLNGKEYKCKVSNKALPAPIEKTISKAKGQPREPQVCTLPPSRDELTKNQVSLSCAVKGFYPSDIAVEWESNGQPENNYKTTPPVLDSDGSFFLVSKLTVDKSRWQQGNVFSCSVMHEALHNHYTQKSLSLSPGK

SEQ ID NO: 209 - protein, 697 aa, synthetic construct
  REGION 1..697: note = hu46H2-F4-1
EVQLVESGGGLVKPGGSLRLSCAASGFTFSNYGMSWVRQAPGKGLEWVSTIGSGGGYTYYSDSVKGRFTISRDNAKNSLYLQMNSLRAEDTAVYYCVRHPQIGYWGQGTLVTVSSASTKGPSVFPLAPSSKSTSGGTAALGCLVKDYFPEPVTVSWNSGALTSGVHTFPAVLQSSGLYSLSSVVTVPSSSLGTQTYICNVNHKPSNTKVDKKVEPKSCEVQLVESGGGLVQPGGSLKLSCAASGFTFNKYAMNWVRQAPGKGLEWVARIRSKYNNYATYYADSVKDRFTISRDDSKNTAYLQMNNLKTEDTAVYYCVRHGNFGNEYISYWAYWGQGTLVTVSSGGGGSGGGGSGGGGSQTVVTQEPSLTVSPGGTVTLTCGSSTGAVTSGNYPNWVQQKPGQAPRGLIGGTKFLAPGTPARFSGSLLGGKAALTLSGVQPEDEAEYYCVLWYSNRWVFGGGTKLTVLGGGDKTHTCPPCPAPEAAGGPSVFLFPPKPKDTLMISRTPEVTCVVVDVSHEDPEVKFNWYVDGVEVHNAKTKPREEQYNSTYRVVSVLTVLHQDWLNGKEYKCKVSNKALPAPIEKTISKAKGQPREPQVYTLPPSRDELTKNQVSLTCLVKGFYPSDIAVEWESNGQPENNYKTTPPVLDSDGSFFLYSKLTVDKSRWQQGNVFSCSVMHEALHNHYTQKSLSLSPGK

SEQ ID NO: 210 - protein, 98 aa, synthetic construct
  REGION 1..98: note = T.0
GIPPKIEALPSDISIDEGKVLTVACAFTGEPTPEVTWSCGGRKIHSQEQGRFHIENTDDLTTLIIMDVQKQDGGLYTLSLGNEFGSDSATVNIHIRSI

SEQ ID NO: 211 - protein, 98 aa, synthetic construct
  REGION 1..98: note = T.1
GIPPKIECLPSDISIDEGKVLTVASAFTGEPTPEVTWSTGGRKIHSQEQGRFHIENTDDLTTLIIMDVQKQDGGLYTLSLGNEFGSDSATVNIHIRSI

SEQ ID NO: 212 - protein, 98 aa, synthetic construct
  REGION 1..98: note = T.2
GIPPKIEALPSDISIDEGKCLTVASAFTGEPTPEVTWSTGGRKIHSQEQGRFHIENTDDLTTLIIMDVQKQDGGLYTLSLGNEFGSDSATVNIHIRSI

SEQ ID NO: 213 - protein, 98 aa, synthetic construct
  REGION 1..98: note = T.3
GIPPKIEALPSDISIDEGKVLTVASCFTGEPTPEVTWSTGGRKIHSQEQGRFHIENTDDLTTLIIMDVQKQDGGLYTLSLGNEFGSDSATVNIHIRSI

SEQ ID NO: 214 - protein, 98 aa, synthetic construct
  REGION 1..98: note = T.4
GIPPKIEALPSDISIDEGKVLCVASAFTGEPTPEVTWSTGGRKIHSQEQGRFHIENTDDLTTLIIMDVQKQDGGLYTLSLGNEFGSDSATVNIHIRSI

SEQ ID NO: 215 - protein, 103 aa, synthetic construct
  REGION 1..103: note = T.5
KAGIRGIPPKIECLPSDISIDEGKVLTVASAFTGEPTPEVTWSTGGRKIHSQEQGRFHIENTDDLTTLIIMDVQKQDGGLYTLSLGNEFGSDSATVNIHIRSI

SEQ ID NO: 216 - protein, 103 aa, synthetic construct
  REGION 1..103: note = T.6
KAGIRGIPPKIEALPSDISIDEGKVLTVACAFTGEPTPEVTWSCGGRKIHSQEQGRFHIENTDDLTTLIIMDVQKQDGGLYTLSLGNEFGSDSATVNIHIRSI

SEQ ID NO: 217 - protein, 98 aa, synthetic construct
  REGION 1..98: note = T.7
GIPPKIECLPSDISIDEGKVLTVASAFTGEPTPEVTWSTGGRKIHSQEQGRFHIENTDDLTTLIISDVQKQDGGLYSLSLGNEFGSDSATVNIHIRSI

SEQ ID NO: 218 - protein, 98 aa, synthetic construct
  REGION 1..98: note = T.8
GIPPKIECLPSDISIDEGKVLTVASAFTGEPTPEVTWSTGGRKIHSQEQGRFHIENTDDLTTLIIKDVQRQDGGLYTLTLRNEFGSDSATVNIHIRSI

SEQ ID NO: 219 - protein, 98 aa, synthetic construct
  REGION 1..98: note = T.9
GIWPKIECLPIDLSIDEGKVLMVASAFTGEPTPEVTWSTGGRKIHSQEQGRFHIENTDDLTTLIIMDVQKQDGGLYTLSLGMEFGSDSATVNIHIRSI

SEQ ID NO: 220 - protein, 98 aa, synthetic construct
  REGION 1..98: note = T.10
GIPPKIECLPIDISIDEGKVLTVASAFTGEPTPEVTWSTGGRKIHSQEQGRFHIENTDDLTTLIIKDVQKQDGGLYTLTLRNEFGSDSATVNIHIRSI

SEQ ID NO: 221 - protein, 98 aa, synthetic construct
  REGION 1..98: note = T.11
GIPPKIECLPSDISIDEGKVLTVASAFTGEPTPEVTWSTSGKKISSEEGGRFHIESTEDLTTLIIMDVQKQDGGVYTLSLGNDLGSDSATVNIHIRSI

SEQ ID NO: 222 - protein, 98 aa, synthetic construct
  REGION 1..98: note = T.12
GIPPKIECLPSDISIDEGKVLTVASAFTGEPTPEVTWSTGGRKIHSEEGGRFHIESTEDLTTLIIMDVQKQDGGVYTLSLGNEFGSDSATVNIHIRSI

SEQ ID NO: 223 - protein, 98 aa, synthetic construct
  REGION 1..98: note = T.13
GIPPKIECLPSDISIDEGKVLTVASAFTGEPTPEVTWSTGGRKIHSQEQGRFHIESTEDLTTLIIMDVQKQDGGVYTLSLGNEFGSDSATVNIHIRSI

SEQ ID NO: 224 - protein, 98 aa, synthetic construct
  REGION 1..98: note = T.14
GIPPKIECLPSDISIDEGKVLTVASAFTGEPTPEVTWSTGGRKIHSQEQGRFHIESTEDLTTLIISDVQKQDGGLYSLSLGNEFGSDSATVNIHIRSI

SEQ ID NO: 225 - protein, 103 aa, synthetic construct
  REGION 1..103: note = T.15
KAGIRGIPPKIECLPSDISIDEGKVLTVASAFTGEPTPEVTWSTGGRKIHSQEQGRFHIESTEDLTTLIISDVQKQDGGLYSLSLGNEFGSDSATVNIHIRSI

SEQ ID NO: 226 - protein, 98 aa, synthetic construct
  REGION 1..98: note = T.16
GIPPKIECLPIDISIDEGKVLTVASAFTGEPTPEVTWSTGGRKIHSQEQGRFHIENTDDSTTLTIKDVQKQDGGLYTLTLRNEFGSDSATVNIHIRSI

SEQ ID NO: 227 - protein, 98 aa, synthetic construct
  REGION 1..98: note = T.17
GIPPKIECLPIDISIDEGKCLTVASAFTGEPTPEVTWSTGGRKIHSQEQGRFHIENTDDSTTLTIKDVQKQDGGLYTLTLRNEFGSDSATVNIHIRSI

SEQ ID NO: 228 - protein, 98 aa, synthetic construct
  REGION 1..98: note = T.18
GIPPKIECLPIDISIDEGKVLTVASCFTGEPTPEVTWSTGGRKIHSQEQGRFHIENTDDSTTLTIKDVQKQDGGLYTLTLRNEFGSDSATVNIHIRSI

SEQ ID NO: 229 - protein, 97 aa, synthetic construct
  REGION 1..97: note = O.0
SGAPRFLTRPKAFVVSVGKDATLSCQIVGNPTPQVSWEKDQQPVAAGARFRLAQDGDLYRLTILDLALGDSGQYVCRARNAIGEAFAAVGLQVDAEA

SEQ ID NO: 230 - protein, 98 aa, synthetic construct
  REGION 1..98: note = OL.0
QGSPPCFLRFPRPVRVVSGAEAELKCVVLGEPPPVVVWEKGGQQLAASERLSFPADGAEHGLLLTAALPTDAGVYVCRARNAAGEAYAAAAVTVLEPP

SEQ ID NO: 231 - protein, 97 aa, synthetic construct
  REGION 1..97: note = O.1
SGAPRFLTRPKAFVVSVGKDATLSCQIVGNPTPQVSWEKDQQPVAAGARFRLAQDGDLYRLTILDLALGDSGQYVCRARNAIGEAFACVGLQVDAEA

SEQ ID NO: 232 - protein, 97 aa, synthetic construct
  REGION 1..97: note = O.2
SGCPRFLTRPKAFVVSVGKDATLSCQIVGNPTPQVSWEKDQQPVAAGARFRLAQDGDLYRLTILDLALGDSGQYVCRARNAIGEAFAAVGLQVDAEA

SEQ ID NO: 233 - protein, 97 aa, synthetic construct
  REGION 1..97: note = O.3
SGAPRFLTCPKAFVVSVGKDATLSCQIVGNPTPQVSWEKDQQPVAAGARFRLAQDGDLYRLTILDLALGDSGQYVCRARNAIGEAFAAVGLQVDAEA

SEQ ID NO: 234 - protein, 97 aa, synthetic construct
  REGION 1..97: note = O.4
SGAPRFLTRPKAFVVSVGKDATLSSQIVGNPTPQVSWEKDQQPVAAGARFRLAQDGDLYRLTILDLALGDSGQYVSRARNAIGEAFACVGLQVDAEA

SEQ ID NO: 235 - protein, 97 aa, synthetic construct
  REGION 1..97: note = O.5
SGCPRFLTRPKAFVVSVGKDATLSSQIVGNPTPQVSWEKDQQPVAAGARFRLAQDGDLYRLTILDLALGDSGQYVSRARNAIGEAFAAVGLQVDAEA

SEQ ID NO: 236 - protein, 97 aa, synthetic construct
  REGION 1..97: note = O.6
SGAPRFLTCPKAFVVSVGKDATLSSQIVGNPTPQVSWEKDQQPVAAGARFRLAQDGDLYRLTILDLALGDSGQYVSRARNAIGEAFAAVGLQVDAEA

SEQ ID NO: 237 - protein, 97 aa, synthetic construct
  REGION 1..97: note = O.7
SGAPRFKTRPKAFVVSVGKDATLSSQIVGNPTPQVSWEKDQQPVAAGARFRLAQDGDLYRLKILDLALGDSGQYVSRARNAIGEAFACVGLQVDAEA

SEQ ID NO: 238 - protein, 97 aa, synthetic construct
  REGION 1..97: note = O.8
SGAPRFKTRPKAFVVSVGKDATLSSQIVGNPTPQVSWEKDQQPVAAGARFRLAQDGDLYRLHILDLALGDSGQYVSRARNAIGEAFACVGLQVDAEA

SEQ ID NO: 239 - protein, 97 aa, synthetic construct
  REGION 1..97: note = O.9
SGAPRFLTRPLAFVVSVGKDATLSSQIVGNPTPQVSWEKDQQPVAAGARFRLAQDGDLYRLKILDLALGDSGQYVSRARNAIGEAFACVGLQVDAEA

SEQ ID NO: 240 - protein, 97 aa, synthetic construct
  REGION 1..97: note = O.10
SGAPRFLTRPLAFVVSVGKDATLSSQIVGNPTPQVSWEKDQQPVAAGARFRLAQDGDLYRLHILDLALGDSGQYVSRARNAIGEAFACVGLQVDAEA

SEQ ID NO: 241 - protein, 102 aa, synthetic construct
  REGION 1..102: note = O.11
DQPQFSGAPRFLTRPKAFVVSVGKDATLSSQIVGNPTPQVSWEKDQQPVAAGARFRLAQDGDLYRLTILDLALGDSGQYVSRARNAIGEAFACVGLQVDAEA

SEQ ID NO: 242 - protein, 102 aa, synthetic construct
  REGION 1..102: note = O.12
DQPQFSGAPRFKTRPKAFVVSVGKDATLSSQIVGNPTPQVSWEKDQQPVAAGARFRLAQDGDLYRLKILDLALGDSGQYVSRARNAIGEAFACVGLQVDAEA

SEQ ID NO: 243 - protein, 102 aa, synthetic construct
  REGION 1..102: note = O.13
DQPQFSGAPRFKTRPKAFVVSVGKDATLSSQIVGNPTPQVSWEKDQQPVAAGARFRLAQDGDLYRLHILDLALGDSGQYVSRARNAIGEAFACVGLQVDAEA

SEQ ID NO: 244 - protein, 102 aa, synthetic construct
  REGION 1..102: note = O.14
DQPQFSGAPRFRTRPKAFVVSVGKDATLSSQIVGNPTPQVSWEKDQQPVAAGARFRLAQDGDLYRLKILDLALGDSGQYVSRARNAIGEAFACVGLQVDAEA

SEQ ID NO: 245 - protein, 102 aa, synthetic construct
  REGION 1..102: note = O.15
DQPQFSGAPRFRTRPKAFVVSVGKDATLSSQIVGNPTPQVSWEKDQQPVAAGARFRLAQDGDLYRLHILDLALGDSGQYVSRARNAIGEAFACVGLQVDAEA

SEQ ID NO: 246 - protein, 102 aa, synthetic construct
  REGION 1..102: note = O.16
DQPQFSGAPRFLTRPKAFVVSVGKDATLSCQIVGNPTPQVSWEKDQQPVAAGARFRLAQDGDLYRLTILDLALGDSGQYVCRARNAIGEAFAAVGLQVDAEA

SEQ ID NO: 247 - protein, 98 aa, synthetic construct
  REGION 1..98: note = OL.1
QGSPPEFLRFPRPVRVVSGAEAELKCVVLGEPPPVVVWEKGGQQLAASERLSFPADGAEHGLLLTAALPTDAGCYVCRARNAAGEAYAAAAVTVLEPP

SEQ ID NO: 248 - protein, 98 aa, synthetic construct
  REGION 1..98: note = OL.2
QGSPPEFLRFPRPVRVVSGAEAELKCVVLGEPPPVVVWEKGGQQLAASERLSFPADGAEHGLLLTAALPTDAGVYVCRARNAACEAYAAAAVTVLEPP

SEQ ID NO: 249 - protein, 98 aa, synthetic construct
  REGION 1..98: note = OL.3
QGSPPEFLRFPRPVRVVSGAEAELKCVVLGEPPPVVVWEKGGQQLAASERLSFPADGAEHGLLLTAALPTDAGVYVCRARNAAGECYAAAAVTVLEPP

SEQ ID NO: 250 - protein, 98 aa, synthetic construct
  REGION 1..98: note = OL.4
QGSPPEFLRFPRPVRVVSGAEAELKSVVLGEPPPVVVWEKGGQQLAASERLSFPADGAEHGLLLTAALPTDAGCYVSRARNAAGEAYAAAAVTVLEPP

SEQ ID NO: 251 - protein, 98 aa, synthetic construct
  REGION 1..98: note = OL.5
QGSPPEFLRFPRPVRVVSGAEAELKSVVLGEPPPVVVWEKGGQQLAASERLSFPADGAEHGLLLTAALPTDAGVYVSRARNAACEAYAAAAVTVLEPP

SEQ ID NO: 252 - protein, 98 aa, synthetic construct
  REGION 1..98: note = OL.6
QGSPPEFLRFPRPVRVVSGAEAELKSVVLGEPPPVVVWEKGGQQLAASERLSFPADGAEHGLLLTAALPTDAGVYVSRARNAAGECYAAAAVTVLEPP

SEQ ID NO: 253 - protein, 97 aa, synthetic construct
  REGION 1..97: note = O.17
SGAPRFLTRPKSYTVSVGKDASLSSQIVGNPTPQVSWEKDQQPVAAGARFRLAQDGDLYRLKILDLALGDSGQYVSRARNAIGEAFACVGLQVDAEA

SEQ ID NO: 254 - protein, 97 aa, synthetic construct
  REGION 1..97: note = O.18
SEAPRFLTRPLAFVVSEGKDATLSSQIVGDPPPEVTWEKDQQPITAGARFRLAQDGDVYRLEILDLQLSDSGQYVSRARNAIGEAFACVGLQVDAEG

SEQ ID NO: 255 - protein, 97 aa, synthetic construct
  REGION 1..97: note = O.19
SGAPRFLTRPLAFVVSVGKLAMLSSQIVGNPTPQVSWEKDQQPVAAGARFRLLQDGDLYRLKILDLALGDSGQYVSRARNAIGEAFACVGLQVDAEA

SEQ ID NO: 256 - protein, 97 aa, synthetic construct
  REGION 1..97: note = O.20
SGAPRFLTRPLAFVVSVGKDATLSSQIVGNPTPQVSWEKDKQPVTAGARFRLAQDGDLYRLKILDLQLSDSGQYVSRARNAIGEAFACLGLQVDAEA

SEQ ID NO: 257 - protein, 97 aa, synthetic construct
  REGION 1..97: note = O.21
SGAPRFLTRPLAFVVSVGKDATLSSQIVGNPTPQVSWEKDQLPVTAGARFRLAQDGDLYRLKILDLTLSDSGQYVSRARNAIGEAFACVGLEVGAEA

SEQ ID NO: 258 - protein, 97 aa, synthetic construct
  REGION 1..97: note = O.22
SGAPRFLTRPLSYVVSVGKDASLSSQIVGNPTPQVSWEKDQLPVTAGARFRLAQDGDLYRLKILDLQLSDSGQYVSRARNAIGEAFACVGLEVGAEA

SEQ ID NO: 259 - protein, 102 aa, synthetic construct
  REGION 1..102: note = O.23
DQPQFSGAPRFLTRPLSYVVSVGKDASLSSQIVGNPTPQVSWEKDQLPVTAGARFRLAQDGDLYRLKILDLQLSDSGQYVSRARNAIGEAFACVGLEVGAEA

SEQ ID NO: 260 - protein, 97 aa, synthetic construct
  REGION 1..97: note = O.24
SGAPRFLTRPKAFVVSVGKDATLSSQIVGNPFPQVSWEKDKQPVTAGVRFRLAQDGDLYRLKILDLQLSDSGQYVSRARNAIGEAFACLGLQVDAEA

SEQ ID NO: 261 - protein, 97 aa, synthetic construct
  REGION 1..97: note = O.25
SGAPRFLTRPKASVVSVGKDATLSSQIVGNPFPQVSWEKDKQPVTAGVRFRLAQDGDLYRLKILDLQLSDSGQYVSRARNAHGEAFACLGLQVDAEA

SEQ ID NO: 262 - protein, 97 aa, synthetic construct
  REGION 1..97: note = O.26
SGCPRFLTRPKASVVSVGKDATLSSQIVGNPFPQVSWEKDKQPVTAGVRFRLAQDGDLYRLKILDLQLSDSGQYVSRARNAHGEAFACLGLQVDAEA

SEQ ID NO: 263 - protein, 97 aa, synthetic construct
  REGION 1..97: note = O.27
SGAPRFLTCPKASVVSVGKDATLSSQIVGNPFPQVSWEKDKQPVTAGVRFRLAQDGDLYRLKILDLQLSDSGQYVSRARNAHGEAFACLGLQVDAEA

SEQ ID NO: 264 - protein, 97 aa, synthetic construct
  REGION 1..97: note = O.28
SGAPRFLTRPKASVVSVGKDATLSCQIVGNPFPQVSWEKDKQPVTAGVRFRLAQDGDLYRLKILDLQLSDSGQYVCRARNAHGEAFACLGLQVDAEA

SEQ ID NO: 265 - protein, 97 aa, synthetic construct
  REGION 1..97: note = O.29
SGCPRFLTRPKASVVSVGKDATLSCQIVGNPFPQVSWEKDKQPVTAGVRFRLAQDGDLYRLKILDLQLSDSGQYVCRARNAHGEAFACLGLQVDAEA

SEQ ID NO: 266 - protein, 97 aa, synthetic construct
  REGION 1..97: note = O.30
SGAPRFLTCPKASVVSVGKDATLSCQIVGNPFPQVSWEKDKQPVTAGVRFRLAQDGDLYRLKILDLQLSDSGQYVCRARNAHGEAFACLGLQVDAEA

SEQ ID NO: 267 - protein, 97 aa, synthetic construct
  REGION 1..97: note = O.31
SGAPRFLTRPKASVVSVGKDATLSSQIVGNPFPQVSWEKDKQPVTAGVRFRLAQDGDLYRLKILDCQLSDSGQYVSRARNAHGEAFACLGLQCDAEA

SEQ ID NO: 268 - protein, 97 aa, synthetic construct
  REGION 1..97: note = O.32
SGCPRFLTRPKASVVSVGKDATLSSQIVGNPFPQVSWEKDKQPVTAGVRFRLAQDGDLYRLKILDCQLSDSGQYVSRARNAHGEAFACLGLQCDAEA

SEQ ID NO: 269 - protein, 97 aa, synthetic construct
  REGION 1..97: note = O.33
SGAPRFLTCPKASVVSVGKDATLSSQIVGNPFPQVSWEKDKQPVTAGVRFRLAQDGDLYRLKILDCQLSDSGQYVSRARNAHGEAFACLGLQCDAEA

SEQ ID NO: 270 - protein, 5 aa, synthetic construct
  REGION 1..5: note = linker
ASTKG

SEQ ID NO: 271 - protein, 5 aa, synthetic construct
  REGION 1..5: note = linker
RTVAS

SEQ ID NO: 272 - protein, 227 aa, synthetic construct
  REGION 1..227: note = Fc1
DKTHTCPPCPAPEAAGGPSVFLFPPKPKDTLMISRTPEVTCVVVDVSHEDPEVKFNWYVDGVEVHNAKTKPREEQYNSTYRVVSVLTVLHQDWLNGKEYKCKVSNKALPAPIEKTISKAKGQPREPQVYTLPPCREEMTKNQVSLWCLVKGFYPSDIAVEWESNGQPENNYKTTPPVLDSDGSFFLYSKLTVDKSRWQQGNVFSCSVMHEALHNHYTQKSLSLSPGK

SEQ ID NO: 273 - protein, 227 aa, synthetic construct
  REGION 1..227: note = Fc2
DKTHTCPPCPAPEAAGGPSVFLFPPKPKDTLMISRTPEVTCVVVDVSHEDPEVKFNWYVDGVEVHNAKTKPREEQYNSTYRVVSVLTVLHQDWLNGKEYKCKVSNKALPAPIEKTISKAKGQPREPQVCTLPPSREEMTKNQVSLSCAVKGFYPSDIAVEWESNGQPENNYKTTPPVLDSDGSFFLVSKLTVDKSRWQQGNVFSCSVMHEALHNHYTQKSLSLSPGK

SEQ ID NO: 274 - protein, 118 aa, synthetic construct
  REGION 1..118: note = VH2-L
QVQLVESGGGVVQPGRSLRLSCAASGFTFSSYTMHWVRQAPGKGLEWVTFISYDGNNKYYADSVKGRFTISRDNSKNTLYLQMNSLRAEDTAIYYCARTGWLGPFDYWGQGTLVTVSS

SEQ ID NO: 275 - protein, 108 aa, synthetic construct
  REGION 1..108: note = VL2-L
EIVLTQSPGTLSLSPGERATLSCRASQSVGSSYLAWYQQKPGQAPRLLIYGAFSRATGIPDRFSGSGSGTDFTLTISRLEPEDFAVYYCQQYGSSPWTFGQGTKVEIK

SEQ ID NO: 276 - protein, 4 aa, synthetic construct
  REGION 1..4: note = linker
GGGS

SEQ ID NO: 277 - protein, 119 aa, synthetic construct
  REGION 1..119: note = hu73H1
EVQLVQSGAEVKKPGSSVKVSCKASGYAFSTSWMNWVRQAPGQGLEWMGRIYPGDGDTKYNGKFQGRVTITADKSTSTAYMELSSLRSEDTAVYYCVRSIYYLYYFDYWGQGTTVTVSS

SEQ ID NO: 278 - protein, 119 aa, synthetic construct
  REGION 1..119: note = hu73H2
EVQLVQSGAEVKKPGSSVKVSCKASGYAFSTSWMNWVRQAPGQGLEWMGRIYPGDGDTKYNGKFQGRVTLTADKSTSTAYMELSSLRSEDTAVYYCVRSIYYLYYFDYWGQGTTVTVSS

SEQ ID NO: 279 - protein, 119 aa, synthetic construct
  REGION 1..119: note = hu73H3
EVQLVQSGAEVKKPGSSVKVSCKASGYAFSTSWMNWVREAPGKGLEWMGRIYPGDGDTKYNGKFQGRVTLTADKSTSTAYMELSSLRSEDTAVYYCVRSIYYLYYFDYWGQGTTVTVSS

SEQ ID NO: 280 - protein, 107 aa, synthetic construct
  REGION 1..107: note = hu73L1
DIQMTQSPSSLSASVGDRVTITCSTSQDIYNNLSWFQQKPGKVPKLLIYYTSSLHSGVPSRFSGSGSGTDYTLTISSLQPEDVATYYCQQYNNLPFTFGGGTKVEIK

SEQ ID NO: 281 - protein, 107 aa, synthetic construct
  REGION 1..107: note = hu73L2
DIQMTQSPSSLSASVGDRVTITCSTSQDIYNNLSWFQQKPGKVVRLLIYYTSSLHSGVPSRFSGSGSGTDYTLTISSLQPEDVATYYCQQYNNLPFTFGGGTKVEIK

SEQ ID NO: 282 - protein, 107 aa, synthetic construct
  REGION 1..107: note = hu73L3
DIQMTQSPSSLSASVGDRVTITCSTSQDIYNNLSWFQQKPDGVVRLLIYYTSSLHSGVPSRFSGSGSGTDYTLTISSLQPEDVATYYCQQYNNLPFTFGGGTKVEIK

SEQ ID NO: 283 - protein, 107 aa, synthetic construct
  REGION 1..107: note = hu73L4
DIQMTQSPSSLSASVGDRVTITCSTSQDIYNNLSWFQQKPDGTVRLLIYYTSSLHSGVPSRFSGSGSGTDYTLTISSLQPEDVATYYCQQYNNLPFTFGGGTKVEIK

SEQ ID NO: 284 - protein, 449 aa, synthetic construct
  REGION 1..449: note = 73VH-F1-1
QVQLQQSGPELVKPGASVKISCKASGYAFSTSWMNWVKERPGKGLEWIGRIYPGDGDTKYNGKFQGKATLTADKSSSTAYMKLSSLTSEDSAVYFCVRSIYYLYYFDYWGQGTTLTVSSASTKGPSVFPLAPSSKSTSGGTAALGCLVKDYFPEPVTVSWNSGALTSGVHTFPAVLQSSGLYSLSSVVTVPSSSLGTQTYICNVNHKPSNTKVDKKVEPKSCDKTHTCPPCPAPEAAGGPSVFLFPPKPKDTLMISRTPEVTCVVVDVSHEDPEVKFNWYVDGVEVHNAKTKPREEQYNSTYRVVSVLTVLHQDWLNGKEYKCKVSNKALPAPIEKTISKAKGQPREPQVYTLPPCRDELTKNQVSLWCLVKGFYPSDIAVEWESNGQPENNYKTTPPVLDSDGSFFLYSKLTVDKSRWQQGNVFSCSVMHEALHNHYTQKSLSLSPGK

SEQ ID NO: 285 - protein, 214 aa, synthetic construct
  REGION 1..214: note = 73VL-CL
DIQMTQPTSSLSASLGDRVTISCSTSQDIYNNLSWFQQKPDGTVRLLIYYTSSLHSGVPSRFSGSGSGTDYSLTISNLEPEDIATYYCQQYNNLPFTFGGGTNLEIRRTVAAPSVFIFPPSDEQLKSGTASVVCLLNNFYPREAKVQWKVDNALQSGNSQESVTEQDSKDSTYSLSSTLTLSKADYEKHKVYACEVTHQGLSSPVTKSFNRGEC

SEQ ID NO: 286 - protein, 677 aa, synthetic construct
  REGION 1..677: note = 73VH-F3-1
QVQLQQSGPELVKPGASVKISCKASGYAFSTSWMNWVKERPGKGLEWIGRIYPGDGDTKYNGKFQGKATLTADKSSSTAYMKLSSLTSEDSAVYFCVRSIYYLYYFDYWGQGTTLTVSSASTKGPSVFPLAPSSKSTSGGTAALGCLVKDYFPEPVTVSWNSGALTSGVHTFPAVLQSSGLYSLSSVVTVPSSSLGTQTYICNVNHKPSNTKVDKKVEPKSCEVQLVESGGGLVQPGGSLKLSCAASGFTFNKYAMNWVRQAPGKGLEWVARIRSKYNNYATYYADSVKDRFTISRDDSKNTAYLQMNNLKTEDTAVYYCVRHGNFGNEYISYWAYWGQGTLVTVSSGGGGSGIPPKIECLPIDISIDEGKVLTVASAFTGEPTPEVTWSTGGRKIHSQEQGRFHIENTDDSTTLTIKDVQKQDGGLYTLTLRNEFGSDSATVNIHIRSIDKTHTCPPCPAPEAAGGPSVFLFPPKPKDTLMISRTPEVTCVVVDVSHEDPEVKFNWYVDGVEVHNAKTKPREEQYNSTYRVVSVLTVLHQDWLNGKEYKCKVSNKALPAPIEKTISKAKGQPREPQVYTLPPSRDELTKNQVSLTCLVKGFYPSDIAVEWESNGQPENNYKTTPPVLDSDGSFFLYSKLTVDKSRWQQGNVFSCSVMHEALHNHYTQKSLSLSPGK